European Patent Specification EP 3 666 797 B1, published May 17, 2023. Title: ANTIGEN BINDING PROTEINS TO PROPROTEIN CONVERTASE SUBTILISIN KEXIN TYPE (PCSK9). Applicant: Jackson, Simon Mark Walker, Nigel P.C. Piper, Derek E. Shan, Bei Shen, Wenyan Chan, Joyce Chi Yee King, Chadwick Terence Ketchem, Randal Robert Mehlin, Christopher Carabeo, Teresa Cao, Qiong. The sequence listing filed with the application follows.

SEQUENCE LISTING (499 sequences)

SEQ ID NO: 1 - protein, 662 aa, Homo sapiens
QEDEDGDYEELVLALRSEEDGLAEAPEHGTTATFHRCAKDPWRLPGTYVVVLKEETHLSQSERTARRLQAQAARRGYLTKILHVFHGLLPGFLVKMSGDLLELALKLPHVDYIEEDSSVFAQSIPWNLERITPPRYRADEYQPPDGGSLVEVYLLDTSIQSDHREIEGRVMVTDFENVPEEDGTRFHRQASKCDSHGTHLAGVVSGRDAGVAKGASMRSLRVLNCQGKGTVSGTLIGLEFIRKSQLVQPVGPLVVLLPLAGGYSRVLNAACQRLARAGVVLVTAAGNFRDDACLYSPASAPEVITVGATNAQDQPVTLGTLGTNFGRCVDLFAPGEDIIGASSDCSTCFVSQSGTSQAAAHVAGIAAMMLSAEPELTLAELRQRLIHFSAKDVINEAWFPEDQRVLTPNLVAALPPSTHGAGWQLFCRTVWSAHSGPTRMATAIARCAPDEELLSCSSFSRSGKRRGERMEAQGGKLVCRAHNAFGGEGVYAIARCCLLPQANCSVHTAPPAEASMGTRVHCHQQGHVLTGCSSHWEVEDLGTHKPPVLRPRGQPNQCVGHREASIHASCCHAPGLECKVKEHGIPAPQGQVTVACEEGWTLTGCSALPGTSHVLGAYAVDNTCVVRSRDVSTTGSTSEEAVTAVAICCRSRHLAQASQELQ

SEQ ID NO: 2 - DNA, 2076 bp, Homo sapiens
atgggcaccgtcagctccaggcggtcctggtggccgctgccactgctgctgctgctgctgctgctcctgggtcccgcgggcgcccgtgcgcaggaggacgaggacggcgactacgaggagctggtgctagccttgcgctccgaggaggacggcctggccgaagcacccgagcacggaaccacagccaccttccaccgctgcgccaaggatccgtggaggttgcctggcacctacgtggtggtgctgaaggaggagacccacctctcgcagtcagagcgcactgcccgccgcctgcaggcccaggctgcccgccggggatacctcaccaagatcctgcatgtcttccatggccttcttcctggcttcctggtgaagatgagtggcgacctgctggagctggccttgaagttgccccatgtcgactacatcgaggaggactcctctgtctttgcccagagcatcccgtggaacctggagcggattacccctccgcggtaccgggcggatgaataccagccccccgacggaggcagcctggtggaggtgtatctcctagacaccagcatacagagtgaccaccgggaaatcgagggcagggtcatggtcaccgacttcgagaatgtgcccgaggaggacgggacccgcttccacagacaggccagcaagtgtgacagtcatggcacccacctggcaggggtggtcagcggccgggatgccggcgtggccaagggtgccagcatgcgcagcctgcgcgtgctcaactgccaagggaagggcacggttagcggcaccctcataggcctggagtttattcggaaaagccagctggtccagcctgtggggccactggtggtgctgctgcccctggcgggtgggtacagccgcgtcctcaacgccgcctgccagcgcctggcgagggctggggtcgtgctggtcaccgctgccggcaacttccgggacgatgcctgcctctactccccagcctcagctcccgaggtcatcacagttggggccaccaatgcccaggaccagccggtgaccctggggactttggggaccaactttggccgctgtgtggacctctttgccccaggggaggacatcattggtgcctccagcgactgcagcacctgctttgtgtcacagagtgggacatcacaggctgctgcccacgtggctggcattgcagccatgatgctgtctgccgagccggagctcaccctggccgagttgaggcagagactgatccacttctctgccaaagatgtcatcaatgaggcctggttccctgaggaccagcgggtactgacccccaacctggtggccgccctgccccccagcacccatggggcaggttggcagctgttttgcaggactgtgtggtcagcacactcggggcctacacggatggccacagccatcgcccgctgcgccccagatgaggagctgctgagctgctccagtttctccaggagtgggaagcggcggggcgagcgcatggaggcccaagggggcaagctggtctgccgggcccacaacgcttttgggggtgagggtgtctacgccattgccaggtgctgcctgctaccccaggccaactgcagcgtccacacagctccaccagctgaggccagcatggggacccgtgtccactgccaccaacagggccacgtcctcacaggctgcagctcccactgggaggtggaggaccttggcacccacaagccgcctgtgctgaggccacgaggtcagcccaaccagtgcgtgggccacagggaggccagcatccacgcttcctgctgccatgccccaggtctggaatgcaaagtcaaggagcatggaatcccggcccctcaggggcaggtgaccgtggcctgcgaggagggctggaccctgactggctgcagcgccctccctgggacctcccacgtcctgggggcctacgccgtagacaacacgtgtgtagtcaggagccgggacgtcagcactacaggcagcaccagcgaagaggccgtgacagccgttgccatctgctgccggagccggcacctggcgcaggcctcccaggagctccag

SEQ ID NO: 3 - protein, 692 aa, Homo sapiens
MGTVSSRRSWWPLPLLLLLLLLLGPAGARAQEDEDGDYEELVLALRSEEDGLAEAPEHGTTATFHRCAKDPWRLPGTYVVVLKEETHLSQSERTARRLQAQAARRGYLTKILHVFHGLLPGFLVKMSGDLLELALKLPHVDYIEEDSSVFAQSIPWNLERITPPRYRADEYQPPDGGSLVEVYLLDTSIQSDHREIEGRVMVTDFENVPEEDGTRFHRQASKCDSHGTHLAGVVSGRDAGVAKGASMRSLRVLNCQGKGTVSGTLIGLEFIRKSQLVQPVGPLVVLLPLAGGYSRVLNAACQRLARAGVVLVTAAGNFRDDACLYSPASAPEVITVGATNAQDQPVTLGTLGTNFGRCVDLFAPGEDIIGASSDCSTCFVSQSGTSQAAAHVAGIAAMMLSAEPELTLAELRQRLIHFSAKDVINEAWFPEDQRVLTPNLVAALPPSTHGAGWQLFCRTVWSAHSGPTRMATAIARCAPDEELLSCSSFSRSGKRRGERMEAQGGKLVCRAHNAFGGEGVYAIARCCLLPQANCSVHTAPPAEASMGTRVHCHQQGHVLTGCSSHWEVEDLGTHKPPVLRPRGQPNQCVGHREASIHASCCHAPGLECKVKEHGIPAPQGQVTVACEEGWTLTGCSALPGTSHVLGAYAVDNTCVVRSRDVSTTGSTSEEAVTAVAICCRSRHLAQASQELQ

SEQ ID NO: 4 - protein, 112 aa, Homo sapiens
DIVMTQSPLSLPVTPGEPASISCRSSQSLLHSNGYNYLDWYLQKPGQSPQLLIYLGSNRASGVPDRFSGSGSGTDFTLKISRVEAEDVGVYYCMQALQTPFTFGPGTKVDIK

SEQ ID NO: 5 - protein, 112 aa, Homo sapiens
DIVMTQSPLSLSVTPGEPPSISCRSSQSLLHSNGYNFLNWYLQKPGQSPQLLIYLGSHRASGVPDRFSGSGSGTDFTLEISRVEAEDVGVYYCMQVLQTPFTFGPGTKVDIK

SEQ ID NO: 6 - protein, 107 aa, Homo sapiens [sequence omitted]

SEQ ID NO: 7 - protein, 107 aa, Homo sapiens
DIQMTQSPSSLSASVGDRVTITCRASQRISNYLSWYLQKPGIAPKLLIYAASSLQSGVPSRFSGSGSGTDFTLTISSLQSEDFATYYCQQSYSTPLIFGGGTKVEIK

SEQ ID NO: 8 - protein, 107 aa, Homo sapiens
DIQMTQSPSSLSASVGDRVTITCRASQSISSYLNWYQQKPGKAPKLLIYAASSLQSGVPSRFSGSGSGTDFTLTISSLQPEDFATYYCQQSYSTPITFGQGTRLEIK

SEQ ID NO: 9 - protein, 107 aa, Homo sapiens
DILMTQSPSSLSASVGDRVTITCRASQSISSYLNWYQQKPGKAPKVLIYAASSLQSGVPSRFSGSGSGTDFTLTINSLQPEDFATYYCQQSYSSPITFGQGTRLEIK

SEQ ID NO: 10 - protein, 107 aa, Homo sapiens
DIQMTQSPSSLSASVGDRVTITCRASQSISIYLNWYQQKPGKAPYLLIYAAASLQSGVPSRFSGSGSGTDFTLTISSLQPEDFATYYCQQSYSAPITFGQGTRLEIK

SEQ ID NO: 11 - protein, 111 aa, Homo sapiens
QSVLTQPPSVSGAPGQRVTISCTGSSSNIGAGYDVHWYQQLPGTAPKLLIYGNSNRPSGVPDRFSGSKSGTSASLAITGLQAEDEADYYCQSYDSSLSGSVFGGGTKLTVL

SEQ ID NO: 12 - protein, 111 aa, Homo sapiens
QSVLTQPPSVSGAPGQRVTISCTGSSSNIGAGYDVHWYQQLPGTAPKLLISGNSNRPSGVPDRFSGSKSGTSASLAITGLQAEDEADYYCQSYDSSLSGSVFGGGTKLTVL

SEQ ID NO: 13 - protein, 111 aa, Homo sapiens
QSVLTQPPSVSGAPGQRVTISCTGSSSNIGAHYDVHWYQQVPGTAPKLLIYGNTYRPSGVPDRFSGSKSGTSASLAITGLQAEDEADYYCQSYDNSLSGVVFGGGTKLTVL

SEQ ID NO: 14 - protein, 108 aa, Homo sapiens
QSALTQPASVSGSPGQSITISCTGTSSDVGGYNYVSWYQQHPGKAPKLMIYEVSNRPSGVSNRFSGSKSGNTASLTISGLQAEDEADYYCSSYTSSSVFGGGTKLTVL

SEQ ID NO: 15 - protein, 109 aa, Homo sapiens
QSALTQPASVSGSPGQSITISCTGTSSDVGRYNSVSWYQHHPGKAPKVMIYEVSNRPSGVSTRFSGSKSGNTASLTISGLQAEDEADYYCSSYTSSSVVFGGGTKLTVL

SEQ ID NO: 16 - protein, 109 aa, Homo sapiens
QSALTQPASVSGSPGQSITISCTGTSSDVGGYNSVSWYQQHPGKPPKLMIYEVSNRPSGVSIRFSGSKSGNTASLTISGLQAEDEADYFCSSYTSTSMVFGGGTKLTVL

SEQ ID NO: 17 - protein, 109 aa, Homo sapiens; identical to SEQ ID NO: 16

SEQ ID NO: 18 - protein, 109 aa, Homo sapiens
QSALTQPASVSGSPGQSITISCTGTSSDVGGYNSVSWYQQHPGKPPKLMIYEVSNRPSGVSNRFSGSKSGNTASLTISGLQAEDEADYFCSSYTSTSMVFGGGTKLAVL

SEQ ID NO: 19 - protein, 109 aa, Homo sapiens
QSALTQPASVSGSPGQSITISCTGTSSDVGGYNSVSWYQQYPGKPPKLKIYEVSNRPSGVSNRFSGSKSGNTASLTISGLQAEDEADYFCSSYTSTSMVFGGGTKLTVL

SEQ ID NO: 20 - protein, 109 aa, Homo sapiens
QSALTQPASVSGSPGQSITISCTGTSSDVGGYNSVSWYQQHPGKPPKLMIYEVSNRPSGVSNRFSGSKSGNTASLTISGLQAEDEADYFCSSYTSTSMVFGGGTKLTVL

SEQ ID NO: 21 - protein, 109 aa, Homo sapiens; identical to SEQ ID NO: 20

SEQ ID NO: 22 - protein, 109 aa, Homo sapiens
QSALTQPASVSGSPGQSITISCTGTNSDVGGYNSVSWYQQHPGKPPKLMIYEVSNRPSGISNRFSGSKSGNTASLTISGLQAEDEADYFCSSYTSTSMVFGGGTKLTVL

SEQ ID NO: 23 - protein, 109 aa, Homo sapiens
QSALTQPASVSGSPGQSITISCTGTSSDVGGYNSVSWYQQHPGKAPKLMIYEVSNRPSGVSNRFSGSKSGNTASLTISGLQAEDEADYYCNSYTSTSMVFGGGTKLTVL

SEQ ID NO: 24 - protein, 109 aa, Homo sapiens
QSALTQPASVSGSPGQSITISCTGTSSDVGAYNSVSWYQQHPGKAPKRMIYEVSNRPSGVSNRFSGSKSGNTASLTISGLQAEDEADYYCSSYTSTNMVFGGGTKLTVL

SEQ ID NO: 25 - protein, 108 aa, Homo sapiens; identical to SEQ ID NO: 14

SEQ ID NO: 26 - protein, 109 aa, Homo sapiens
QSALTQPASVSGSPGQSITISCTGTSSDVGGYNSVSWYQQHPGKAPKLMIYEVTNRPSGVSNRFSGSKSGNTASLTISGLQAEDEADYYCNSYTSTSMVFGGGTKLTVL

SEQ ID NO: 27 - protein, 108 aa, Homo sapiens
QSALTQPASVSGSPGQSITISCTGTSSDVGSYNLVSWYQQHPGKAPKLMIYEGSKRPSGVSNRFSGSKSGNTASLTISGLQAEDEADYYCCSYAGSSTFGGGTKLTVL

SEQ ID NO: 28 - protein, 110 aa, Homo sapiens
LSALTQPASVSGSPGQSITISCTGTSSDVGNYNLVSWYQQYSGKAPKLMIYEVSKRPSGVSNRFSGSKSGNTASLTISGLQAEDEADYYCCSYAGSSTLVFGGGTKLTVL

SEQ ID NO: 29 - protein, 108 aa, Homo sapiens
QSVLTQPPSASGTPGQRVTISCSGSSSNIGSNTVNWYQQLPGTAPKLLIYSNNQRPSGVPDRFSGSKSGTSASLAISGLQSEDEADYYCAAWDDSLNVFGGGTKLTVL

SEQ ID NO: 30 - protein, 109 aa, Homo sapiens
QSVLTQPPSASGTPGQRVTISCSGSSSNIGSKTVNWYQQVPGTAPKLLIYRNNQRPLGVPDRFSGSKSGTSASLAISGLQSEDEADYYCAAWDDSLNWVFGGGTKLTVL

SEQ ID NO: 31 - protein, 109 aa, Homo sapiens
QSVLTQPPSASGPPGQRVTISCSGSSSNIGSNTVNWYQQLPGTAPKLLIYSNNRRPSGVPDRFSGSKSGTSASLAISGLQSEDEADYYCAAWDDSLNWVFGGGTKLTVL

SEQ ID NO: 32 - protein, 110 aa, Homo sapiens
QSVLTQPPSASGTPGQRVTISCSGSSSNIGSNTVNWYQQLPGTAPKLLIYSNNQRPSGVPDRFSGSKSGTSASLAISGLQSEDEADYYCAVWDDSLNGWVFGGGTKLTVL

SEQ ID NO: 33 - protein, 109 aa, Homo sapiens
QSVLTQPPSASGTPGQRVTISCSGSSSNIGSKTVNWYQQFPGTAPKLLIYSNNRRPSGVPDRFSGSKSGTSASLAISGLQSEDEADYYCAAWDDSLNWVFGAGTKLTVL

SEQ ID NO: 34 - protein, 110 aa, Homo sapiens
QSVLTQPPSVSAAPGQKVTISCSGSSSNIGNNYVSWYQQLPGTAPKLLIYDNNKRPSGIPDRFSGSKSGTSATLGITGLQTGDEADYYCGTWDSSLSAYVFGTGTKVTVL

SEQ ID NO: 35 - protein, 110 aa, Homo sapiens
QSVLTQPPSVSAAPGQKVTISCSGSSSNIGNNFVSWYQQLPGTAPKLLIYDYNKRPSGIPDRFSGSKSGTSATLGITGLQTGDEADYYCGTWDSSLSAYVFGTGTRVTVL

SEQ ID NO: 36 - protein, 110 aa, Homo sapiens
QSVLTQPPSVSAAPGQKVTISCSGSSSNIGNNFVSWYQQLPGTAPKLLIYDYNKRPSGIPDRFSGSKSGTSATLGITGLQTGDEADYYCGTWDSSLSGYVFGTGTRVTVL

SEQ ID NO: 37 - protein, 110 aa, Homo sapiens
QSVLTQPPSVSAAPGQKVTISCSGSSSNIGNNFVSWYQQFPGTAPKLLIYDYNKRPSGIPDRFSGSKSGTSATLGITGLQTGDEADYYCGTWDSSLSSYVFGTGTRVTVL

SEQ ID NO: 38 - protein, 110 aa, Homo sapiens; identical to SEQ ID NO: 36

SEQ ID NO: 39 - protein, 110 aa, Homo sapiens
QSVLTQPPTVSAAPGQKVTISCSGSSSNIGNNFVSWYQQLPGTAPKLLIYDYNKRPSGIPDRFSGSKSGTSATLGITGLQTGDEADYYCGTWDSSLSGYVFGTGTRVTVL

SEQ ID NO: 40 - protein, 110 aa, Homo sapiens
QSVLTQPPSVSAAPGQKVTISCSGSSSNIGNNFVSWYQQLPGTAPKLLIYDSNKRPSGIPDRFSGSKSGTSATLDITGLQTGDEADYYCGTWDSSLSAYVFGTGTKVTVL

SEQ ID NO: 41 - protein, 110 aa, Homo sapiens
QSVLTQPPSVSAAPGQKVTISCSGSSSNIGNNYVSWYQQLPGTAPKLLIYDNNKRPSGIPDRFSGSKSGTSATLGITGLQTGDEADYYCGTWDSSLSAVVFGGGTKLTVL

SEQ ID NO: 42 - protein, 110 aa, Homo sapiens
QSVLTQPPSVSAAPGQKVTISCSGSNSNIGNNYVSWYQQLPGTAPKLLIYDNNKRPSGIPDRFSGSNSGTSATLGITGLQTGDEADYYCGTWDSSLSAVVFGGGTKLTVL

SEQ ID NO: 43 - protein, 107 aa, Homo sapiens
SYELTQPPSVSVSPGQTASITCSGDKLGDKYACWYQQKPGQSPVLVIYQDSKRPSGIPERFSGSNSGNTATLTISGTQAMDEADYYCQAWDSSTAVVFGGGTKLTVL

SEQ ID NO: 44 - protein, 106 aa, Homo sapiens
SYELTQPPSVSVSPGQTARITCSGDKLGDKYACWYQQKPGQSPVLVIYQNTKWPLGIPERFSGSKSGNTVTLTISGTQAMDEADYYCQAWDSSTVVFGGGTKLTVL

SEQ ID NO: 45 - protein, 116 aa, Homo sapiens
QPVLTQPPSASASLGASVTLTCTLSSGYSNYKVDWYQQRPGKGPRFVMRVGTGGIVGSKGDGIPDRFSVLGSGLNRYLTIKNIQEEDESDYHCGADHGSGSNFVVVFGGGTKLTVL

SEQ ID NO: 46 - protein, 116 aa, Homo sapiens
QPVLTQPLFASASLGASVTLTCTLSSGYSSYEVDWYQQRPGKGPRFVMRVDTGGIVGSKGEGIPDRFSVLGSGLNRYLTIKNIQEEDESDYHCGADHGSGTNFVVVFGGGTKLTVL

SEQ ID NO: 47 - protein, 114 aa, Homo sapiens
QVQLVQSGAEVKKPGASVKVSCKASGYTFTSYGISWVRQAPGQGLEWMGWISAYNGNTNYAQKLQGRVTMTTDTSTSTAYMELRSLRSDDTAVYYCARYGMDVWGQGTTVTVSS

SEQ ID NO: 48 - protein, 115 aa, Homo sapiens
QIQLVQSGAEVKKPGASVKVSCKASGYPLTSYGISWVRQAPGQGLEWMGWISAYNGNTNYAQKVQGSVTMTTDTSTSTVYMELRSLRSDDTAVYYCARGYGMDVWGQGTTVTVSS

SEQ ID NO: 49 - protein, 115 aa, Homo sapiens
QVQLVQSGAEVKKPGASVKVSCKASGYTLTSYGISWVRQAPGQGLEWMGWVSFYNGNTNYAQKLQGRGTMTTDPSTSTAYMELRSLRSDDTAVYYCARGYGMDVWGQGTTVTVSS

SEQ ID NO: 50 - protein, 115 aa, Homo sapiens; identical to SEQ ID NO: 49

SEQ ID NO: 51 - protein, 115 aa, Homo sapiens
QVQLVQSGAEVKKPGASVKVSCKASGYTLTSYGISWVRQAPGQGLEWMGWISFYNGNTNYAQKVQGRVTMTTDTSTSTVYMELRSLRSDDTAVYYCARGYGMDVWGQGTTVTVSS

SEQ ID NO: 52 - protein, 115 aa, Homo sapiens
QVQLVQSGAEVKRPGASVKVSCKASGYTLTSYGISWVRQAPGQGLEWMGWISVYNGNTNYAQKVQGRVTMTTDTSTSTVYMELRSLSSDDTAVYYCARGYGMDVWGQGTTVTVSS

SEQ ID NO: 53 - protein, 115 aa, Homo sapiens
QIQLVQSGAEVKKPGASVKVSCKASGYTLTSYGISWVRQAPGQGLEWMGWISFYNGNTNYAQKVQGRVTMTTDTSTSTVYMELRSLRSDDTAVYFCARGYGMDVWGQGTTVTVSS

SEQ ID NO: 54 - protein, 115 aa, Homo sapiens
QVQLVQSGAEVKKPGASLKVSCKASGYSLTSYGISWVRQAPGQGLEWMGWISAYNGNTNYAQKVQGRVTMTTDTSTSTVYMEVRSLRSDDTAVYYCARGYGMDVWGQGTTVTVSS

SEQ ID NO: 55 - protein, 115 aa, Homo sapiens
QVQLVQSGAEVKKPGASVKVSCKASGYPLTSYGISWVRQAPGQGLEWMGWISAYNGNTNYAQKVQGRVTMTTDTSTSTVYMELRSLRSDDTAVYYCARGYGMDVWGQGTTVTVSS

SEQ ID NO: 56 - protein, 115 aa, Homo sapiens
QVQLVQSGAEVKKPGASVKVSCKASGYALTSYGISWVRQAPGQGLEWMGWISAYNGNTNYAQKVQGRVTMTTDTSTSTVYMELRSLRSDDTAVYYCARGYGMDVWGQGTTVTVSS

SEQ ID NO: 57 - protein, 115 aa, Homo sapiens
QVQLVQSGAEVKKPGASVKVSCKASGYSFTSYGISWVRQAPGQGLEWMGWVSAYNGNTNYAQKFQGRVTMTTDTSTSTAYMELRSLRSDDTAVYYCARGYVMDVWGQGTTVTVSS

SEQ ID NO: 58 - protein, 115 aa, Homo sapiens
QVQLVQSGAEVKKPGASVKVSCKASGYTFPSYGISWVRQAPGQGLEWMGWISAYNGNTNYAEKLQGRVTMTTDTSTSTAYMEVRSLRSDDTAVFYCARGYVMDVWGQGTTVTVSS

SEQ ID NO: 59 - protein, 113 aa, Homo sapiens
QVQLVQSGAEVKKPGASVKVSCKASGYTFTSYGISWVRQAPGQGLEWMGWISAYNGNTNYAQKLQGRVTMTTDTSTSTAYMELRSLRSDDTAVYYCARGYDYWGQGTLVTVSS

SEQ ID NO: 60 - protein, 115 aa, Homo sapiens
QVQLVQSGAEVKKPGASVKVSCKASGYTFTSYGISWVRQAPGQGLEWMGWISTYNGNTNYAQKVQGRVTMTTDTSTSTAYMELRSLRSDDTAVYYCARGYTRDYWGQGTLVTVSS

SEQ ID NO: 61 - protein, 116 aa, Homo sapiens
EVQLVESGGGLVQPGGSLRLSCAASGFTFSSYWMSWVRQAPGKGLEWVANIKQDGSEKYYVDSVKGRFTISRDNAKNSLYLQMNSLRAEDTAVYYCARNWGAFDVWGQGTMVTVSS

SEQ ID NO: 62 - protein, 119 aa, Homo sapiens
EVQLVESGGGLVQPGGSLRLSCAASGFTFSRYWMSWVRQAPGKGLEWVANIKHDGSEKYYVDSVKGRFTISRDNAKNSLYLQMNSLRAEDTAVYYCARESNWGFAFDVWGHGTMVTVSS

SEQ ID NO: 63 - protein, 116 aa, Homo sapiens
EVQLVESGGGLVQPGGSLRLSCAASGFTFSSYWMSWVRQAPGKGLEWVANIKQDGSEKYYVDSVKGRFTISRDNAKNSLYLQMNSLRAEDTAVYYCARNWGAFDIWGQGTMVTVSS

SEQ ID NO: 64 - protein, 119 aa, Homo sapiens
EVQLVESGGGLVQPGGSLRLSCVVSGFTFSSYWMSWVRQAPGKGLEWVANIKQDGSEKYYVDSVKGRFTISRDNAKNSLYLQMNSLRAEDTAVYYCARESNWGFAFDIWGQGTMVTVSS

SEQ ID NO: 65 - protein, 119 aa, Homo sapiens
EVQLVESGGGLVQPGGSLRLSCAASGLTFSNFWMSWVRQAPGKGLEWVANIKQDGSEKYYVDSVKGRFTISRDNAKNSLYLQMNSLRAEDTAVYSCTRESNWGFAFDIWGQGTMVTVSS

SEQ ID NO: 66 - protein, 123 aa, Homo sapiens
EVQLVESGGGLVKPGGSLRLSCAASGFTFSSYSMNWVRQAPGKGLEWVSSISSSSSYIYYADSVKGRFTISRDNAKNSLYLQMNSLRAEDTAVYYCARDYDFWSGYYTAFDVWGQGTMVTVSS

SEQ ID NO: 67 - protein, 123 aa, Homo sapiens
EVQLVESGGGLVKPGGSLRLSCAASGFTFSSYSMNWVRQAPGKGLEWVSSISSSSSYISYADSVKGRFTISRDNAKNSLYLQMNSLRAEDTAVYFCARDYDFWSAYYDAFDVWGQGTMVTVSS

SEQ ID NO: 68 - protein, 112 aa, Homo sapiens
EVQLLESGGGLVQPGGSLRLSCAASGFTFSSYAMSWVRQAPGKGLEWVSAISGSGGSTYYADSVKGRFTISRDNSKNTLYLQMNSLRAEDTAVYYCAKFDYWGQGTLVTVSS

SEQ ID NO: 69 - protein, 117 aa, Homo sapiens
EVQLLESGGGLVQPGGSLRLSCAASGFTFSSYAMSWVRQAPGKGLEWVSTISGSGGRTYYADSVKGRFTISRDNSKNTLYLQMNSLRAEDTAVYYCAKEVGSPFDYWGQGTLVTVSS

SEQ ID NO: 70 - protein, 117 aa, Homo sapiens
EVQLLESGGGLVQPGGSLRLSCAASGFTFSSYAMSWVRQAPGKGLEWVSAISGSGGSTYYADSVKGRFTISRDNSKNTLYLQMNSLRAEDTAVYYCAKVLMVYADYWGQGTLVTVSS

SEQ ID NO: 71 - protein, 121 aa, Homo sapiens
EVQLLESGGGLVQPGGSLRLSCAASGFTFSSYAMNWVRQAPGKGLEWVSTISGSGDNTYYADSVKGRFTISRDNSKNTLYLQMNSLRAEDTAVYYCAKKFVLMVYAMLDYWGQGTLVTVSS

SEQ ID NO: 72 - protein, 121 aa, Homo sapiens
EVQLLESGGGLVQPGGSLRLSCAASGFTFSSYAMNWVRQAPGKGLEWVSTISGSGGNTYYADSVKGRFTISRDNSKNTLYLQMNSLRAEDTAVYYCAKKFVLMVYAMLDYWGQGTLVTVSS

SEQ ID NO: 73 - protein, 116 aa, Homo sapiens
QVQLVESGGGVVQPGRSLRLSCAASGFTFSSYGMHWVRQAPGKGLEWVAVIWYDGSNKYYADSVKGRFTISRDNSKNTLYLQMNSLRAEDTAVYYCARYYYGMDVWGQGTTVTVSS

SEQ ID NO: 74 - protein, 123 aa, Homo sapiens
QVQLVESGGGVVQPGRSLRLSCAASGFTFSSYGMHWVRQAPGKGLEWVAVIWYDGSDKYYADSVKGRFTISRDNSKNTLYLQMNSLRAEDTAVYYCARETGPLKLYYYGMDVWGQGTTVTVSS

SEQ ID NO: 75 - protein, 116 aa, Homo sapiens
QVQLVESGGGVVQPGRSLRLSCAASGFTFSSYGMHWVRQAPGKGLEWVAVIWYDGSNKYYADSVKGRFTISRDNSKNTLYLQMNSLRAEDTAVYYCARIAAGMDVWGQGTTVTVSS

SEQ ID NO: 76 - protein, 122 aa, Homo sapiens
QVHLVESGGGVVQPGRSLRLSCAASGFTFNSFGMHWVRQAPGKGLEWVALIWSDGSDKYYADSVKGRFTISRDNSKNTLYLQMNSLRAEDTAVYYCARAIAALYYYYGMDVWGQGTTVTVSS

SEQ ID NO: 77 - protein, 122 aa, Homo sapiens
QVQLVESGGGVVQPGRSLRLSCAASGFTFSSFGMHWVRQAPGKGLEWVALIWNDGSNKYYADSVKGRFTISRDNSKNTLYLQMNSLRAEDTAVYYCARAIAALYYYYGMDVWGHGTTVTVSS

SEQ ID NO: 78 - protein, 122 aa, Homo sapiens
QVQLVESGGGVVQPGRSLRLSCAASGFTFSSFGMHWVRQAPGKGLEWVALIWNDGSNKYYADSVKGRFTISRDNSKNTLYLQMNSLRAEDTAVYYCARAIAALYYYYGMDVWGQGTTVTVSS

SEQ ID NO: 79 - protein, 122 aa, Homo sapiens
QVHLVESGGGVVQPGRSLRLSCAASGFTFNSFGMHWVRQAPGKGLEWVALIWSDGSDEYYADSVKGRFTISRDNSKNTLYLQMNSLRAEDTAVYYCARAIAALYYYYGMDVWGQGTTVTVSS

SEQ ID NO: 80 - protein, 122 aa, Homo sapiens; identical to SEQ ID NO: 78

SEQ ID NO: 81 - protein, 122 aa, Homo sapiens
QVQLVESGGGVVQPGRSLRLSCAASGFTFSSYGMHWVRQAPGKGLEWVAIIWYDGSNKYYADSVKGRFTISRDNSKNTLYLQMNSLRAEDTAVYYCARRGGLAARPGGMDVWGQGTTVTVSS

SEQ ID NO: 82 - protein, 122 aa, Homo sapiens
QVQLVESGGGVVQPGRSLRLSCAASGFTFSSYGMHWVRQAPGKGLEWVAVIWYDGSNKYYADSVKGRFTISRDNSKNTLYLQMNSLRAEDTAVYYCARGIAVAYYYYGMDVWGQGTTVTVSS

SEQ ID NO: 83 - protein, 122 aa, Homo sapiens
QVQLVESGGGVVQPGRSLRLSCAASGFTFRSYGMHWVRQAPGKGLEWVALIWHDGSNTYYVDSVKGRFTISRDNSKNTLYLQMNSLRAEDTAVYYCARGIAVAYYYYGMDVWGQGTTVTVSS

SEQ ID NO: 84 - protein, 117 aa, Homo sapiens
QVQLQESGPGLVKPSQTLSLTCTVSGGSISSGGYYWSWIRQHPGKGLEWIGYIYYSGSTYYNPSLKSRVTISVDTSKNQFSLKLSSVTAADTAVYYCARYYYGMDVWGQGTTVTVSS

SEQ ID NO: 85 - protein, 122 aa, Homo sapiens
QVQLQESGPGLVKPSQTLSLTCTVSGGSISSSDYYWSWIRQHPGKGLEWIGYIYYSGSTYYNPSLKSRITISVDTSKNLFSLKLSSVTAADTAVYYCARGGVTTYYYAMDVWGQGTTVTVSS

SEQ ID NO: 86 - protein, 120 aa, Homo sapiens
QVQLQESGPGLVKPSQTLSLTCTVSGGSISSGGYYWSWIRQHPGKGLEWIGYIYYSGSTYYNPSLKSRVTISVDTSKNQFSLKLSSVTAADTAVYYCAREDTAMVYFDYWGQGTLVTVSS

SEQ ID NO: 87 - protein, 121 aa, Homo sapiens
QVQLQESGPGLVKPSQTLSLTCTVSGGSISSGGYYWSWIRQHPGKGLEWIGYIYNSGSTYYNPSLKSRVTISVDTSKNQFSLKLSSVTAADTAVYYCAREDTAMVPYFDYWGQGTLVTVSS

SEQ ID NO: 88 - protein, 115 aa, Homo sapiens
QVQLQQWGAGLLKPSETLSLTCAVYGGSFSGYYWSWIRQPPGKGLEWIGEINHSGSTNYNPSLKSRVTISVDTSKNQFSLKLSSVTAADTAVYYCARGQLVFDYWGQGTLVTVSS

SEQ ID NO: 89 - protein, 116 aa, Homo sapiens
QVQLQQWGAGLLKPSETLSLTCAVYGGSFSAYYWNWIRQPPGKGLEWIGEINHSGRTDYNPSLKSRVTISVDTSKKQFSLKLNSVTAADTAVYYCARGQLVPFDYWGQGTLVTVSS

SEQ ID NO: 90 - protein, 115 aa, Homo sapiens
QVQLQQSGPGLVKPSQTLSLTCAISGDSVSSNSAAWNWIRQSPSRGLEWLGRTYYRSKWYNDYAVSVKSRITINPDTSKNQFSLQLNSVTPEDTAVYYCARFDYWGQGTLVTVSS

SEQ ID NO: 91 - protein, 121 aa, Homo sapiens
QVQLQQSGPGLVKPSQTLSLTCAISGDSVSSNSAAWNWIRQSPSRGLEWLGRTYYRSKWYKNYSVSVKSRITINPDTSKNQFSLQLNSVTPGDTAVYYCARGGPTAAFDYWGQGTLVTVSS

SEQ ID NO: 92 - DNA, 345 bp, Homo sapiens
cagattcagctggtgcagtctggagctgaggtgaagaagcctggggcctcagtgaaggtctcctgcaaggcttctggttaccccttgaccagctatggtatcagctgggtgcgacaggcccctggacaagggcttgagtggatgggatggatcagcgcttacaatggtaacacaaactatgcacagaaggtccagggcagcgtcaccatgaccacagacacatccacgagcacagtctacatggagctgaggagcctgagatctgacgacacggccgtgtattactgtgcgagaggctacggtatggacgtctggggccaagggaccacggtcaccgtctcctct

SEQ ID NO: 93 - DNA, 327 bp, Homo sapiens
cagtctgccctgactcagcctgcctccgtgtctgggtctcctggacagtcgatcaccatctcctgcactggaaccagcagtgacgttggtggttataactctgtctcctggtaccaacagtacccaggcaaaccccccaaactcaagatttatgaggtcagtaatcggccctcaggggtttctaatcgcttctctggctccaagtctggcaacacggcctccctgaccatctctgggctccaggctgaggacgaggctgattatttctgcagctcatatacaagcaccagcatggtcttcggcggagggaccaagctgaccgtccta

SEQ ID NO: 94 - DNA, 345 bp, Homo sapiens
caggttcagctggtgcagtctggagctgaggtgaagaagcctggggcctcagtgaaggtctcctgcaaggcttctggttacaccttaaccagctatggtatcagctgggtgcgacaggcccctggacaagggcttgagtggatgggatgggtcagtttttataatggtaacacaaactatgcacagaagctccagggcagaggcaccatgaccacagacccatccacgagcacagcctacatggagctgaggagcctgagatctgacgacacggccgtgtattactgtgcgagaggctacggtatggacgtctggggccaagggaccacggtcaccgtctcctct

SEQ ID NO: 95 - DNA, 327 bp, Homo sapiens
cagtctgccctgactcagcctgcctccgtgtctgggtctcctggacagtcgatcaccatctcctgcactggaaccagcagtgacgttggtggttataactctgtctcctggtaccaacagcacccaggcaaagcccccaaactcatgatttatgaggtcagtaatcggccctcaggggtttctaatcgcttctctggctccaagtctggcaacacggcctccctgaccatctctgggctccaggctgaggacgaggctgattattactgcaattcatatacaagcaccagcatggtattcggcggagggaccaagctgaccgtccta

SEQ ID NO: 96 - DNA, 345 bp, Homo sapiens
caggttcagctggtgcagtctggagctgaagtgaagaagcctggggcctcagtgaaggtctcctgcaaggcttctggttacaccttgaccagctatggtatcagctgggtgcgacaggcccctggacaagggcttgagtggatgggatggatcagcttttacaatggtaacacaaactatgcacagaaggtccagggcagagtcaccatgaccacagacacatccacgagcacagtctacatggagctgaggagcctgagatctgacgacacggccgtgtattactgtgcgagaggctacggtatggacgtctggggccaagggaccacggtcaccgtctcctct

SEQ ID NO: 97 - DNA, 327 bp, Homo sapiens
cagtctgccctgactcagcctgcctccgtgtctgggtctcctggacagtcgatcaccatctcctgcactggaaccagcagtgacgttggtggttataactctgtctcctggtaccaacagcacccaggcaaaccccccaaactcatgatttatgaggtcagtaatcggccctcaggggtttctattcgcttctctggctccaagtctggcaacacggcctccctgaccatctctgggctccaggctgaggacgaggctgattatttctgcagctcatatacaagcaccagcatggtcttcggcggagggaccaagctgaccgtccta

SEQ ID NO: 98 - DNA, 345 bp, Homo sapiens
cagattcagctggtgcagtctggagctgaggtgaagaagcctggggcctcagtgaaggtctcctgcaaggcttctggttacaccttgaccagctatggtatcagctgggtgcgacaggcccctggacaagggcttgagtggatgggatggatcagcttttacaatggtaacacaaactatgcacagaaggtccagggcagagtcaccatgaccacagacacatccacgagcacagtctacatggagctgaggagcctgagatctgacgacacggccgtgtatttctgtgcgagaggttacggtatggacgtctggggccaagggaccacggtcaccgtctcctca

SEQ ID NO: 99 - DNA, 327 bp, Homo sapiens
cagtctgccctgactcagcctgcctccgtgtctgggtctcctggacagtcgatcaccatctcctgcactggaaccagcagtgacgttggtggttataactctgtctcgtggtaccaacagcacccaggcaaaccccccaaactcatgatttatgaggtcagtaatcggccctcaggggtttctaatcgcttctctggctccaagtctggcaacacggcctccctgaccatctctgggctccaggctgaggacgaggctgattatttctgcagctcatatacaagcaccagcatggtcttcggcggagggaccaagctggccgtccta

SEQ ID NO: 100 - DNA, 345 bp, Homo sapiens
caggttcagctggtgcagtctggagctgaggtgaagaagcctggggcctcagtgaaggtctcctgcaaggcttctggttacaccttaaccagctatggtatcagctgggtgcgacaggcccctggacaagggcttgagtggatgggatgggtcagtttttataatggtaacacaaactatgcacagaagctccagggcagaggcaccatgaccacagacccatccacgagcacagcctacatggagctgaggagcctgagatctgacgacacggccgtgtattactgtgcgagaggctacggtatggacgtctggggccaagggaccacggtcaccgtctcctca

SEQ ID NO: 101 - DNA, 327 bp, Homo sapiens
cagtctgccctgactcagcctgcctccgtgtctgggtctcctggacagtcgatcaccatctcctgcactggaaccagcagtgacgttggtggttataactctgtctcctggtaccaacagcacccaggcaaagcccccaaactcatgatttatgaggtcactaatcggccctcaggggtttctaatcgcttctctggctccaagtctggcaacacggcctccctgaccatctctgggctccaggctgaggacgaggctgattattactgcaactcatatacaagcaccagcatggtgttcggcggagggaccaagctgaccgtccta

SEQ ID NO: 102 - DNA, 363 bp, Homo sapiens
caggtgcagctgcaggagtcgggcccaggactggtgaagccttcacagaccctgtccctcacctgcactgtctctggtggctccatcagcagtggtggttactactggagctggatccgccagcacccagggaagggcctggagtggattgggtacatatataacagtgggagcacctactacaacccgtccctcaagagtcgagttaccatatcagtagacacgtctaagaaccagttctccctgaagctgagctctgtgactgccgcggacacggccgtgtattactgtgcgagagaggatacagctatggttccttactttgactactggggccagggaaccctggtcaccgtctcctca

SEQ ID NO: 103 - DNA, 333 bp, Homo sapiens
cagtctgtactgacgcagccgccctcagtgtctggggccccagggcagagggtcaccatctcctgcactgggagcagctccaacatcggggcacattatgatgtgcactggtaccagcaggttccaggaacagcccccaaactcctcatctatggtaacacctatcggccctcaggggtccctgaccgattctctggctccaagtctggcacctcagcctccctggccatcactgggctccaggctgaggatgaggctgattattactgccagtcctatgacaacagcctgagtggtgtggtattcggcggagggaccaagctgaccgtccta

SEQ ID NO: 104 - DNA, 366 bp, Homo sapiens
caggtgcacctggtggagtctgggggaggcgtggtccagcctgggaggtccctgagactctcctgtgcagcgtctggattcaccttcaacagctttggcatgcactgggtccgccaggctccaggcaaggggctggagtgggtggcacttatctggtctgatggaagtgatgaatactatgcagactccgtgaagggccgattcaccatctccagagacaattccaagaacacgctgtatctgcaaatgaacagcctgagagccgaggacacggctgtgtattactgtgcgagagccatagcagccctctactactactacggtatggacgtctggggccaagggaccacggtcaccgtctcctca

SEQ ID NO: 105 - DNA, 330 bp, Homo sapiens
cagtctgtgttgacgcagccgccctcagtgtctgcggccccaggacagaaggtcaccatctcctgctctggaagcagctccaacattgggaataattttgtatcctggtaccagcagctcccaggaacagcccccaaactcctcatttatgactataataagcgaccctcagggattcctgaccgattctctggctccaagtctggcacgtcagccaccctgggcatcaccggactccagactggggacgaggccgattattactgcggaacatgggatagcagcctgagtgcttatgtcttcggaactgggaccagggtcaccgtccta

SEQ ID NO: 106 - DNA, 366 bp, Homo sapiens
caggtgcagctggtggagtctgggggaggcgtggtccagcctgggaggtccctgagactctcctgtgcagcgtctggattcaccttcagcagctttggcatgcactgggtccgccaggctccaggcaaggggctggagtgggtggcacttatatggaatgatggaagtaataaatactatgcagactccgtgaagggccgattcaccatctccagagacaattccaagaacacgctgtatctgcaaatgaacagcctgagagccgaggacacggctgtgtattactgtgcgagagccatagcagccctctactactactacggtatggacgtctggggccaagggaccacggtcaccgtctcctca

SEQ ID NO: 107 - DNA, 330 bp, Homo sapiens
cagtctgtgttgacgcagccgccctcagtgtctgcggccccaggacagaaggtcaccatctcctgctctggaagcagctccaacattgggaataattttgtatcctggtaccagcagctcccaggaacagcccccaaactcctcatttatgactataataagcgaccctcagggattcctgaccgattctctggctccaagtctggcacgtcagccaccctgggcatcaccggactccagactggggacgaggccgattattactgcggaacatgggatagcagtctgagtggttatgtcttcggaactgggaccagggtcaccgtccta

SEQ ID NO: 108 - DNA, 366 bp, Homo sapiens
caggtgcacctggtggagtctgggggaggcgtggtccagcctgggaggtccctgagactctcctgtgcagcgtctggattcaccttcaacagctttggcatgcactgggtccgccaggctccaggcaaggggctggagtgggtggcacttatatggtctgatggaagtgataaatactatgcagactccgtgaagggccgattcaccatctccagagacaattccaagaacacgctgtatctgcaaatgaacagcctgagagccgaggacacggctgtgtattactgtgcgagagccatagcagccctctactactactacggtatggacgtctggggccaagggaccacggtcaccgtctcctca

SEQ ID NO: 109 - DNA, 330 bp, Homo sapiens
cagtctgtgttgacgcagccgccctcagtgtctgcggccccaggacagaaggtcaccatctcctgctctggaagcagttccaacattgggaataattttgtatcctggtaccagcagttcccaggaacagcccccaaactcctcatttatgactataataagcgaccctcagggattcctgaccgattctctggctccaagtctggcacgtcagccaccctgggcatcaccggactccagactggggacgaggccgattattactgcggaacatgggatagcagcctgagttcttatgtcttcggaactgggaccagggtcaccgtccta

SEQ ID NO: 110 - DNA, 366 bp, Homo sapiens
caggtgcagctggtggagtctgggggaggcgtggtccagcctgggaggtccctgagactctcctgtgcagcgtctggattcaccttcagcagctttggcatgcactgggtccgccaggctccaggcaaggggctggagtgggtggcacttatatggaatgatggaagtaataaatactatgcagactccgtgaagggccgattcaccatctccagagacaattccaagaacacgctgtatctgcaaatgaacagcctgagagccgaggacacggctgtgtattactgtgcgagagccatagcagccctctactactactacggtatggacgtctggggccacgggaccacggtcaccgtctcctca

SEQ ID NO: 111 - DNA, 330 bp, Homo sapiens
cagtctgtgttgacgcagccgccctcagtgtctgcggccccaggacagaaggtcaccatctcctgctctggaagcagctccaacattgggaataattttgtatcctggtaccagcagctcccaggaacagcccccaaactcctcatttatgactataataagcgaccctcagggattcctgaccgattctctggctccaagtctggcacgtcagccaccctgggcatcaccggactccagactggggacgaggccgattattactgcggaacatgggatagcagcctgagtggttatgtcttcggaactgggaccagggtcaccgtccta

SEQ ID NO: 112 - DNA, 366 bp, Homo sapiens; identical to SEQ ID NO: 106

SEQ ID NO: 113 - DNA, 330 bp, Homo sapiens
cagtctgtgttgacgcagccgcccacagtgtctgcggccccaggacagaaggtcaccatctcctgctctggaagcagctccaacattgggaataattttgtatcctggtaccagcagctcccaggaacagcccccaaactcctcatttatgactataataagcgaccctcagggattcctgaccgattctctggctccaagtctggcacgtcagccaccctgggcatcaccggactccagactggggacgaggccgattactactgcggaacatgggatagcagcctgagtggttatgtcttcggaactgggaccagggtcaccgtccta

SEQ ID NO: 114 - DNA, 366 bp, Homo sapiens
caggtgcagctggtggagtctgggggaggcgtggtccagcctgggaggtccctgagactctcctgtgcagcgtctggattcaccttcaggagctatggcatgcactgggtccgccaggctccaggcaaggggctggagtgggtggcacttatatggcatgatggaagtaatacatactatgtagactccgtgaagggccgattcaccatctccagagacaattccaagaacacgctgtatctgcaaatgaacagcctgagagccgaggacacggctgtgtattactgtgcgagaggtatagcagtggcttactactactacggtatggacgtctggggccaagggaccacggtcaccgtctcctca

SEQ ID NO: 115 - DNA, 330 bp, Homo sapiens
cagtctgtgttgacgcagccgccctcagtgtctgcggccccaggacagaaggtcaccatctcctgctctggaagcagctccaacattgggaataattttgtatcctggtaccagcagctcccaggaacagcccccaaactcctcatttatgacagtaataagcgaccctcagggattcctgaccgattctctggctccaagtctggcacgtcagccaccctggacatcaccggactccagactggggacgaggccgattattactgcggaacatgggatagcagcctgagtgcttatgttttcggaactgggaccaaggtcaccgtccta

SEQ ID NO: 116 - DNA, 363 bp, Homo sapiens
gaggtgcagctgttggagtctgggggaggcttggtacagcctggggggtccctgagactctcctgtgcagcctctggattcacctttagcagctatgccatgaactgggtccgccaggctccagggaaggggctggagtgggtctcaactattagtggtagtggtgataacacatactacgcagactccgtgaagggccggttcaccatctccagagacaattccaagaacacgctgtatctgcaaatgaacagcctgagagccgaggacacggccgtatattactgtgcgaaaaagtttgtactaatggtgtatgctatgcttgactactggggccagggaaccctggtcaccgtctcctca

SEQ ID NO: 117 - DNA, 321 bp, Homo sapiens
gacatcctgatgacccagtctccatcctccctgtctgcatctgttggagacagagtcaccatcacttgccgggcaagtcagagcattagcagttatttaaattggtatcagcagaaaccagggaaagcccctaaggtcctgatctatgctgcctccagtttgcaaagtggggtcccatcaaggttcagtggcagtggatctgggacagatttcactctcaccatcaacagtctgcaacctgaagattttgcaacttactactgtcaacagagttacagttcccccatcaccttcggccaagggacacgactggagattaaa

SEQ ID NO: 118 - DNA, 363 bp, Homo sapiens
gaggtgcagctgttggagtctgggggaggcttggtacagccgggggggtccctgagactctcctgtgcagcctctggattcacctttagcagctatgccatgaactgggtccgccaggctccagggaaggggctggagtgggtctcaactattagtggtagtggtggtaacacatactacgcagactccgtgaagggccggttcaccatctccagagacaattccaagaacacgctgtatctgcaaatgaacagcctgagagccgaggacacggccgtatattactgtgcgaaaaagtttgtactaatggtgtatgctatgcttgactactggggccagggaaccctggtcaccgtctcctca

SEQ ID NO: 119 - DNA, 321 bp, Homo sapiens
gacatccagatgacccagtctccatcctccctatctgcatctgtaggagacagagtcaccatcacttgccgggcaagtcagagcattagcatctatttaaattggtatcagcagaagccagggaaagccccttacctcctgatctatgctgcagccagtttgcaaagtggggtcccatcaaggttcagtggcagtggatctgggacagatttcactctcaccatcagcagtctgcaacctgaagattttgcaacttactactgtcaacagagttacagtgcccccatcaccttcggccaagggacacgactggagattaaa

SEQ ID NO: 120 - DNA, 345 bp, Homo sapiens
caggttcagctggtgcagtctggagctgaggtgaagaagcctggggcctcactgaaggtctcctgcaaggcttctggttacagtttgaccagctatggtatcagctgggtgcgacaggcccctggacaagggcttgagtggatgggatggatcagcgcttacaatggtaacacaaactatgcacagaaggtccagggcagagtcaccatgaccacagacacatccacgagcacagtctacatggaggtgaggagtctgagatctgacgacacggccgtgtattactgtgcgagaggctacggtatggacgtctggggccaagggaccacggtcaccgtctcctca

SEQ ID NO: 121 - DNA, 327 bp, Homo sapiens
cagtctgccctgactcagcctgcctccgtgtctgggtctcctggacagtcgatcaccatctcctgcactggaaccagcagtgacgttggtggttataactctgtctcctggtaccaacagcacccaggcaaaccccccaaactcatgatttatgaggtcagtaatcggccctcaggggtttctaatcgcttctctggctccaagtctggcaatacggcctccctgaccatctctgggctccaggctgaggacgaggctgattatttctgcagctcatatacaagcaccagcatggtcttcggcggagggaccaagctgaccgtccta

SEQ ID NO: 122 - DNA, 345 bp, Homo sapiens
caggttcagctggtgcagtctggagctgaggtgaagaggcctggggcctcagtgaaggtctcctgcaaggcttctggttacaccttgaccagctatggtatcagctgggtgcgacaggcccctggacaagggcttgagtggatgggatggatcagcgtttacaatggtaacacaaactatgcacagaaggtccagggcagagtcaccatgaccacagacacatccacgagcacagtctacatggagctgaggagcctgagctctgacgacacggccgtgtattactgtgcgagaggctacggtatggacgtctggggccaagggaccacggtcaccgtctcctca

SEQ ID NO: 123 - DNA, 327 bp, Homo sapiens; identical to SEQ ID NO: 97

SEQ ID NO: 124 - DNA, 345 bp, Homo sapiens
caggttcagctggtgcagtctggagctgaggtgaagaagcctggggcctcagtgaaggtctcctgcaaggcttctggttaccccttgaccagctatggtatcagctgggtgcgacaggcccctggacaagggcttgagtggatgggatggatcagcgcttacaatggtaacacaaactatgcacagaaggtccagggcagagtcaccatgaccacagacacatccacgagcacagtctacatggagttgaggagcctgagatctgacgacacggccgtgtattactgtgcgagaggctacggtatggacgtctggggccaagggaccacggtcaccgtctcctca

SEQ ID NO: 125 - DNA, 327 bp, Homo sapiens; identical to SEQ ID NO: 121

SEQ ID NO: 126 - DNA, 345 bp, Homo sapiens
caggttcagttggtgcagtctggagctgaggtgaagaagcctggggcctcagtgaaggtctcctgcaaggcttctggttacgccttgaccagctatggtatcagctgggtgcgacaggcccctggacaagggcttgagtggatgggatggatcagcgcttacaatggtaacacaaactatgcacagaaggtccagggcagagtcaccatgaccacagacacatccacgagcacagtctacatggagctgaggagcctgagatctgacgacacggccgtgtattactgtgcgagaggctacggtatggacgtctggggccaagggaccacggtcaccgtctcctca

SEQ ID NO: 127 - DNA, 327 bp, Homo sapiens
cagtctgccctgactcagcctgcctccgtgtctgggtctcctggacagtcgatcaccatctcctgcactggaaccaacagtgacgttggtggttataactctgtctcctggtaccaacagcacccaggcaaaccccccaaactcatgatttatgaggtcagtaatcggccctcagggatttctaatcgcttctctggctccaagtctggcaacacggcctccctgaccatctctgggctccaggctgaggacgaggctgattatttctgcagctcatatacaagcaccagcatggtcttcggcggagggaccaagctgaccgtccta

SEQ ID NO: 128 - DNA, 345 bp, Homo sapiens
caggttcagctggtgcagtctggagctgaggtgaagaagcctggggcctcagtgaaggtctcctgcaaggcttctggttacagctttaccagctatggtatcagctgggtgcgacaggcccctggacaagggcttgagtggatgggatgggtcagcgcttacaatggtaacacaaactatgcacagaagttccagggcagagtcaccatgaccacagacacatccacgagcacagcctacatggaactgaggagcctgagatctgacgacacggccgtgtattactgtgcgagaggctacgttatggacgtctggggccaagggaccacggtcaccgtctcctca

SEQ ID NO: 129 - DNA, 327 bp, Homo sapiens
cagtctgccctgactcagcctgcctccgtttctgggtctcctggacagtcgatcaccatctcctgcactggaaccagcagtgacgttggtgcttataactctgtctcctggtaccaacagcacccaggcaaagcccccaaacgcatgatttatgaggtcagtaatcggccctcaggggtttctaatcgcttctctggctccaagtctggcaacacggcctccctgaccatctctgggctccaggctgaggacgaggctgattattactgcagctcatatacaagcaccaacatggtattcggcggagggaccaagctgaccgtccta

SEQ ID NO: 130 - DNA, 363 bp, Homo sapiens
caggtacagttgcagcagtcaggtccaggactggtgaagccctcgcagaccctctcactcacctgtgccatctccggggacagtgtctctagcaacagtgctgcttggaactggatcaggcagtccccatcgagaggccttgagtggctgggaaggacatactacaggtccaagtggtataaaaattattcagtatctgtgaaaagtcgaataaccatcaacccagacacatccaagaaccagttctctctgcaactgaactctgtgactcccggggacacggctgtgtattactgtgcaagaggggggccaactgctgcttttgactactggggccagggaaccctggtcaccgtctcctca

SEQ ID NO: 131 - DNA, 330 bp, Homo sapiens
ctttctgccctgactcagcctgcctccgtgtctgggtctcctggacagtcgatcaccatctcctgcactggaaccagcagtgatgttgggaattataaccttgtctcctggtaccaacagtattcaggcaaagcccccaaactcatgatttatgaggtcagtaagcggccctcaggggtttctaatcgcttctctggctccaagtctggcaacacggcctccctgacaatctctgggctccaggctgaggacgaggctgattattactgctgctcatatgcaggtagtagcactttggttttcggcggagggaccaagctgaccgtccta

SEQ ID NO: 132 - DNA, 357 bp, Homo sapiens
gaggtgcagttggtggagtctgggggaggcttggtccagcctggggggtccctgagactctcctgtgtagtctctggattcacctttagtagctattggatgagctgggtccgccaggctccagggaaggggctggagtgggtggccaacataaagcaagatggaagtgagaaatactatgtggactctgtgaagggccgattcaccatctccagagacaacgccaagaactcactgtatctgcaaatgaacagcctgagagccgaggacacggctgtatattactgtgcgagagagtcaaactggggatttgcttttgatatctggggccaagggacaatggtcaccgtctcttca

SEQ ID NO: 133 - DNA, 327 bp, Homo sapiens
cagtctgtgctgactcagccaccctcagcgtctgggacccccgggcagagggtcaccatctcttgttctggaagcagctccaacatcggaagtaagactgtaaactggtaccaacaggtcccaggaacggcccccaaactcctcatctataggaataatcagcggcccttaggggtccctgaccgattctctggctccaagtctggcacctcagcctccctggccatcagtgggctccagtctgaggatgaggctgattattattgtgcagcatgggatgacagcctgaattgggtgttcggcggagggaccaagctgaccgtccta

SEQ ID NO: 134 - DNA, 357 bp, Homo sapiens
gaggtgcagctggtggagtctgggggaggcttggtccagcctggggggtccctgagactctcctgtgcagcctctggattcacctttagtcgctattggatgagctgggtccgccaggctccagggaaggggctggagtgggtggccaacataaagcatgatggaagtgagaaatactatgtggactctgtgaagggccgattcaccatttccagagacaacgccaagaactcactgtatctgcaaatgaacagcctgagagccgaggacacggctgtgtattactgtgcgagagagtcaaactggggatttgcttttgatgtctggggccacgggacaatggtcaccgtctcttca

SEQ ID NO: 135 - DNA, 327 bp, Homo sapiens
cagtctgtgctgactcagccaccctcagcgtctgggccccccggacagagggtcaccatctcttgttctggaagcagctccaacatcggaagtaatactgtaaactggtaccagcagctcccaggaacggcccccaaactcctcatctatagtaataatcggcggccctcaggggtccctgaccgattctctggctccaagtctggcacctcagcctccctggccatcagtgggctccagtctgaggatgaggctgattattactgtgcagcatgggatgacagcctgaattgggtgttcggcggagggaccaagctgaccgtccta

SEQ ID NO: 136 - DNA, 351 bp, Homo sapiens
gaggtgcagctgttggagtctgggggaggcttggtacagcctggggggtccctgagactctcctgtgcagcctctggattcacctttagcagctatgccatgagctgggtccgccaggctccagggaaggggctggagtgggtctcaactattagtggtagtggtggtaggacatattacgcagactccgtgaagggccggttcaccatctccagagacaattccaagaacacgctgtatctgcaaatgaacagcctgagagccgaggacacggccgtatattactgtgcgaaagaagttggcagtccctttgactactggggccagggaaccctggtcaccgtctcctca

SEQ ID NO: 137 - DNA, 330 bp, Homo sapiens
cagtctgtgttgacgcagccgccctcagtgtctgcggccccaggacagaaggtcaccatctcctgctctggaagcaactccaacattgggaataattatgtatcctggtaccagcagctcccaggaacagcccccaaactcctcatttatgacaataataagcgaccctcagggattcctgaccgattctctggctccaactctggcacgtcagccaccctgggcatcaccggactccagactggggacgaggccgattattactgcggaacatgggatagcagcctgagtgctgtggtattcggcggagggaccaagctgaccgtccta

SEQ ID NO: 138 - DNA, 366 bp, Homo sapiens
caggtgcagctggtggagtctgggggaggcgtggtccagcctgggaggtccctgagactctcctgtgcagcgtctggattcaccttcagtagctatggcatgcactgggtccgccaggctccaggcaaggggctggagtgggtggcaattatatggtatgatggaagtaataaatactatgcagactccgtgaagggccgattcaccatctccagagacaattccaagaacacactgtatcttcaaatgaacagcctgagagccgaggacacggctgtgtattactgtgcgaggagggggggtctggcagctcgtccgggcggtatggacgtctggggccaagggaccacggtcaccgtctcctca

SEQ ID NO: 139 - DNA, 318 bp, Homo sapiens
tcctatgagctgactcagccaccctcagtgtctgtgtccccaggacagacagccagaatcacctgctctggagataaattgggggataaatatgcttgctggtatcagcagaaaccaggccagtcccctgtgctggtcatctatcaaaataccaagtggcccttagggatccctgagcgattctctggctccaagtctgggaacacagtcactctgaccatcagcgggacccaggctatggatgaggctgactattactgtcaggcgtgggacagcagcactgtggtattcggcggagggaccaagctgaccgtccta

SEQ ID NO: 140 - DNA, 366 bp, Homo sapiens
caggtgcagctgcaggagtcgggcccaggactggtgaagccttcacagaccctgtccctcacctgcactgtctctggtggctccatcagcagtagtgattactactggagctggatccgccagcacccagggaagggcctggagtggattgggtacatctattacagtgggagcacctactacaacccgtccctcaagagtcgaattaccatatcagtagacacgtctaagaacctgttctccctgaagttgagctctgtgactgccgcggacacggccgtgtattactgtgcgagagggggggtgactacgtactactacgctatggacgtctggggccaagggaccacggtcaccgtctcctca

SEQ ID NO: 141 - DNA, 321 bp, Homo sapiens
gacatacagatgacccagtctccatcctccctgtctgcatctgtaggagacagagtcaccatcacttgccgggcaagtcagcgcattagcaactatttaagttggtatctgcagaaaccagggattgcccctaagctcctgatctatgctgcatccagtttgcagagtggggtcccatcaaggttcagtggcagtggatctgggacagatttcactctcaccatcagcagtctgcaatctgaagattttgcaacttactactgtcaacagagttacagtaccccgctcattttcggcggagggaccaaggtggagatcaaa

SEQ ID NO: 142 - DNA, 369 bp, Homo sapiens
caggtgcagctggtggagtctgggggaggcgtggtccagcctgggaggtccctgagactctcctgtgcagcgtctggattcaccttcagtagctatggcatgcactgggtccgccaggctccaggcaaggggctggagtgggtggcagttatatggtatgatggaagtgataaatactatgcagactccgtgaagggccgattcaccatctccagagacaattccaagaacacgctgtatctgcaaatgaacagcctgagagccgaggacacggctgtgtattactgtgcgagagagactggtcccttgaaactctactactacggtatggacgtctggggccaagggaccacggtcaccgtctcctca

SEQ ID NO: 143 - DNA, 336 bp, Homo sapiens
gatattgtgatgactcagtctccactctccctgtccgtcacccctggagagccgccctccatctcctgcaggtctagtcagagcctcctgcatagtaatggatacaactttttgaattggtacctgcagaagccagggcagtctccacaactcctgatctatttgggttctcatcgggcctccggggtccctgacaggttcagtggcagtggatcaggcacagattttacactggaaatcagcagagtggaggctgaggatgttggggtttattactgcatgcaagttctacaaactccattcactttcggccctgggaccaaagtggatatcaaa

SEQ ID NO: 144 - DNA, 357 bp, Homo sapiens
gaggtgcagctggtggagtctgggggaggcttggtccagcctggggggtccctgagactctcctgtgcagcctctggactcacctttagtaacttttggatgagctgggtccgccaggctccagggaaggggctggagtgggtggccaacataaagcaagatggaagtgagaaatactatgtggactctgtgaagggccgattcaccatctccagagacaacgccaagaattcactgtatctgcaaatgaacagcctgagagccgaggacacggctgtgtattcctgtacgagagagtcaaactggggatttgcttttgatatctggggccaagggacaatggtcaccgtctcttca

SEQ ID NO: 145 - DNA, 327 bp, Homo sapiens
cagtctgtgctgactcagccaccctcagcgtctgggacccccgggcagagggtcaccatctcttgttctggaagcagctccaacatcggaagtaaaactgtaaactggtaccagcagttcccaggaacggcccccaaactcctcatctatagtaataatcggcggccctcaggggtccctgaccgattctctggctccaagtctggcacctcagcctccctggccatcagtgggctccagtctgaggatgaggctgattattactgtgcagcatgggatgacagcctgaattgggtgttcggcgcagggaccaagctgaccgtccta

SEQ ID NO: 146 - DNA, 345 bp, Homo sapiens
caggttcagctggtgcagtctggagctgaggtgaagaagcctggggcctcagtgaaggtctcctgcaaggcttctggttacacctttaccagctatggtatcagctgggtgcgacaggcccctggacaagggcttgagtggatgggatggatcagcacttacaatggtaacacaaactatgcacagaaggtccagggcagagtcaccatgaccacagacacatccacgagcacagcctacatggagctgaggagcctgagatctgacgacacggccgtttattactgtgcgagagggtatactcgggactactggggccagggaaccctggtcaccgtctcctca

SEQ ID NO: 147 - DNA, 348 bp, Homo sapiens
cagcctgtgctgactcagccactttttgcatcagcctccctgggagcctcggtcacactcacctgcaccctgagcagcggctacagtagttatgaagtggactggtatcagcagagaccagggaagggcccccggtttgtcatgcgagtggacactggtgggattgtgggatccaagggggaaggcatccctgatcgcttctcagttttgggctcaggcctgaatcggtatctgaccatcaagaacatccaggaagaggatgagagtgactaccactgtggggcagaccatggcagtgggaccaacttcgtggtggtattcggcggagggaccaagctgaccgtccta

SEQ ID NO: 148 - DNA, 348 bp, Homo sapiens
caggtgcagctacagcagtggggcgcaggactgttgaagccttcggagaccctgtccctcacctgcgctgtctatggtgggtccttcagtgcgtactactggaactggatccgccagcccccagggaaggggctggagtggattggggaaatcaatcatagtggaagaaccgactacaacccgtccctcaagagtcgagtcaccatatcagtagacacgtccaagaagcagttctccctgaagctgaactctgtgaccgccgcggacacggctgtgtattactgtgcgagagggcagctcgtcccctttgactactggggccagggaaccctggtcaccgtctcttca

SEQ ID NO: 149 - DNA, 330 bp, Homo sapiens
cagtctgtgctgactcagccaccctcagcgtctgggacccccgggcagagggtcaccatctcttgttctggaagcagctccaacatcggaagtaatactgtaaattggtatcagcaactcccaggaacggcccccaaactcctcatctatagtaataatcagcggccctcaggggtccctgaccgattctctggctccaagtctggcacctcagcctccctggccatcagtgggctccagtctgaggatgaggctgattattactgtgcagtatgggatgacagcctgaatggttgggtgttcggcggagggaccaagctgaccgtccta

SEQ ID NO: 150 - DNA, 345 bp, Homo sapiens
caggttcagctggtgcagtctggagctgaggtgaagaagcctggggcctcagtgaaggtctcctgcaaggcttctggttacacctttcccagctatggtatcagctgggtgcgacaggcccctggacaagggcttgagtggatgggatggatcagcgcttacaatggtaacacaaactatgcagagaagctccagggcagagtcaccatgaccacagacacatccacgagcacagcctacatggaggtgaggagcctgagatctgacgacacggccgtgttttactgtgcgagaggctacgttatggacgtctggggccaagggaccacggtcaccgtctcctct

SEQ ID NO: 151 - DNA, 327 bp, Homo sapiens
cagtctgccctgactcagcctgcctccgtgtctgggtctcctggacagtcgatcaccatctcctgcactggaaccagcagtgacgttggtcgttataattctgtctcctggtaccaacaccacccaggcaaagcccccaaagtcatgatttatgaggtcagtaatcggccctcaggggtttctactcgcttctctggctccaagtctggcaacacggcctccctgaccatctctgggctccaggctgaggacgaggctgattattactgcagctcatatacaagcagcagcgttgtattcggcggagggaccaaactgaccgtccta

SEQ ID NO: 152 - DNA, 369 bp, Homo sapiens
gaggtgcagctggtggagtctgggggaggcctggtcaagcctggggggtccctgagactctcctgtgcagcctctggattcaccttcagtagctatagcatgaactgggtccgccaggctccagggaaggggctggagtgggtctcatccattagtagtagtagtagttacatttcctacgcagactcagtgaagggccgattcaccatctccagagacaacgccaagaactcactgtatctgcaaatgaacagcctgagagccgaggacacggctgtgtatttctgtgcgagagattacgatttttggagtgcttactatgatgcttttgatgtctggggccaagggacaatggtcaccgtctcttca

SEQ ID NO: 153 - DNA, 333 bp, Homo sapiens
cagtctgtgctgacgcagccgccctcagtgtctggggccccagggcagagggtcaccatctcctgcactgggagcagctccaacatcggggcaggttatgatgtacactggtaccagcagcttccaggaacagcccccaaactcctcatctctggtaacagcaatcggccctcaggggtccctgaccgattctctggctccaagtctggcacctcagcctccctggccatcactgggctccaggctgaggatgaggctgattattactgccagtcctatgacagcagcctgagtggttcggtattcggcggagggaccaagctgaccgtccta

SEQ ID NO: 154 - protein, 326 aa, Homo sapiens
ASTKGPSVFPLAPCSRSTSESTAALGCLVKDYFPEPVTVSWNSGALTSGVHTFPAVLQSSGLYSLSSVVTVPSSNFGTQTYTCNVDHKPSNTKVDKTVERKCCVECPPCPAPPVAGPSVFLFPPKPKDTLMISRTPEVTCVVVDVSHEDPEVQFNWYVDGVEVHNAKTKPREEQFNSTFRVVSVLTVVHQDWLNGKEYKCKVSNKGLPAPIEKTISKTKGQPREPQVYTLPPSREEMTKNQVSLTCLVKGFYPSDIAVEWESNGQPENNYKTTPPMLDSDGSFFLYSKLTVDKSRWQQGNVFSCSVMHEALHNHYTQKSLSLSPGK

SEQ ID NO: 155 - protein, 327 aa, Homo sapiens
ASTKGPSVFPLAPCSRSTSESTAALGCLVKDYFPEPVTVSWNSGALTSGVHTFPAVLQSSGLYSLSSVVTVPSSSLGTKTYTCNVDHKPSNTKVDKRVESKYGPPCPSCPAPEFLGGPSVFLFPPKPKDTLMISRTPEVTCVVVDVSQEDPEVQFNWYVDGVEVHNAKTKPREEQFNSTYRVVSVLTVLHQDWLNGKEYKCKVSNKGLPSSIEKTISKAKGQPREPQVYTLPPSQEEMTKNQVSLTCLVKGFYPSDIAVEWESNGQPENNYKTTPPVLDSDGSFFLYSRLTVDKSRWQEGNVFSCSVMHEALHNHYTQKSLSLSLGK

SEQ ID NO: 156 - protein, 105 aa, Homo sapiens
QPKAAPSVTLFPPSSEELQANKATLVCLISDFYPGAVTVAWKADSSPVKAGVETTTPSKQSNNKYAASSYLSLTPEQWKSHRSYSCQVTHEGSTVEKTVAPTECS

SEQ ID NO: 157 - protein, 106 aa, Homo sapiens
TVAAPSVFIFPPSDEQLKSGTASVVCLLNNFYPREAKVQWKVDNALQSGNSQESVTEQDSKDSTYSLSSTLTLSKADYEKHKVYACEVTHQGLSSPVTKSFNRGEC

SEQ ID NO: 158 - protein, 14 aa, Homo sapiens
TGTSSDVGGYNSVS

SEQ ID NO: 159 - protein, 14 aa, Homo sapiens
TGTNSDVGGYNSVS

SEQ ID NO: 160 - protein, 14 aa, Homo sapiens
TGTSSDVGAYNSVS

SEQ ID NO: 161 - protein, 14 aa, Homo sapiens
TGTSSDVGRYNSVS

SEQ ID NO: 162 - protein, 7 aa, Homo sapiens
EVSNRPS

SEQ ID NO: 163 - protein, 7 aa, Homo sapiens
EVTNRPS

SEQ ID NO: 164 - protein, 9 aa, Homo sapiens
SSYTSTSMV

SEQ ID NO: 165 - protein, 9 aa, Homo sapiens
NSYTSTSMV

SEQ ID NO: 166 - protein, 9 aa, Homo sapiens
SSYTSTNMV

SEQ ID NO: 167 - protein, 9 aa, Homo sapiens
SSYTSSSVV

SEQ ID NO: 168 - protein, 10 aa, Homo sapiens
GYPLTSYGIS

SEQ ID NO: 169 - protein, 10 aa, Homo sapiens
GYSLTSYGIS

SEQ ID NO: 170 - protein, 10 aa, Homo sapiens
GYALTSYGIS

SEQ ID NO: 171 - protein, 10 aa, Homo sapiens
GYTLTSYGIS

SEQ ID NO: 172 - protein, 10 aa, Homo sapiens
GYSFTSYGIS

SEQ ID NO: 173 - protein, 10 aa, Homo sapiens
GYTFPSYGIS

SEQ ID NO: 174 - protein, 17 aa, Homo sapiens
WISAYNGNTNYAQKVQG

SEQ ID NO: 175 - protein, 17 aa, Homo sapiens
WVSFYNGNTNYAQKLQG

SEQ ID NO: 176 - protein, 17 aa, Homo sapiens
WISFYNGNTNYAQKVQG

SEQ ID NO: 177 - protein, 17 aa, Homo sapiens
WISVYNGNTNYAQKVQG

SEQ ID NO: 178 - protein, 17 aa, Homo sapiens
WVSAYNGNTNYAQKFQG

SEQ ID NO: 179 - protein, 17 aa, Homo sapiens
WISAYNGNTNYAEKLQG

SEQ ID NO: 180 - protein, 6 aa, Homo sapiens
GYGMDV

SEQ ID NO: 181 - protein, 6 aa, Homo sapiens
GYVMDV

SEQ ID NO: 182 - protein, 13 aa, Homo sapiens
SGSSSNIGNNFVS

SEQ ID NO: 183 - protein, 7 aa, Homo sapiens
DYNKRPS

SEQ ID NO: 184 - protein, 7 aa, Homo sapiens
DSNKRPS

SEQ ID NO: 185 - protein, 11 aa, Homo sapiens
GTWDSSLSGYV

SEQ ID NO: 186 - protein, 11 aa, Homo sapiens
GTWDSSLSAYV

SEQ ID NO: 187 - protein, 11 aa, Homo sapiens
GTWDSSLSSYV

SEQ ID NO: 188 - protein, 10 aa, Homo sapiens
GFTFSSFGMH

SEQ ID NO: 189 - protein, 10 aa, Homo sapiens
GFTFNSFGMH

SEQ ID NO: 190 - protein, 10 aa, Homo sapiens
GFTFRSYGMH

SEQ ID NO: 191 - protein, 17 aa, Homo sapiens
LIWNDGSNKYYADSVKG

SEQ ID NO: 192 - protein, 17 aa, Homo sapiens
LIWSDGSDEYYADSVKG

SEQ ID NO: 193 - protein, 17 aa, Homo sapiens
LIWSDGSDKYYADSVKG

SEQ ID NO: 194 - protein, 17 aa, Homo sapiens
LIWHDGSNTYYVDSVKG

SEQ ID NO: 195 - protein, 13 aa, Homo sapiens
AIAALYYYYGMDV

SEQ ID NO: 196 - protein, 13 aa, Homo sapiens
GIAVAYYYYGMDV

SEQ ID NO: 197 - protein, 13 aa, Homo sapiens
SGSSSNIGSNTVN

SEQ ID NO: 198 - protein, 13 aa, Homo sapiens
SGSSSNIGSKTVN

SEQ ID NO: 199 - protein, 7 aa, Homo sapiens
SNNRRPS

SEQ ID NO: 200 - protein, 7 aa, Homo sapiens
RNNQRPL

SEQ ID NO: 201 - protein, 10 aa, Homo sapiens
AAWDDSLNWV

SEQ ID NO: 202 - protein, 10 aa, Homo sapiens
GFTFSRYWMS

SEQ ID NO: 203 - protein, 10 aa, Homo sapiens
GLTFSNFWMS

SEQ ID NO: 204 - protein, 10 aa, Homo sapiens
GFTFSSYWMS

SEQ ID NO: 205 - protein, 17 aa, Homo sapiens
NIKHDGSEKYYVDSVKG

SEQ ID NO: 206 - protein, 17 aa, Homo sapiens
NIKQDGSEKYYVDSVKG

SEQ ID NO: 207 - protein, 10 aa, Homo sapiens
ESNWGFAFDV

SEQ ID NO: 208 - protein, 10 aa, Homo sapiens
ESNWGFAFDI

SEQ ID NO: 209 - protein, 11 aa, Homo sapiens
RASQSISSYLN

SEQ ID NO: 210 - protein, 11 aa, Homo sapiens
RASQSISIYLN

SEQ ID NO: 211 - protein, 7 aa, Homo sapiens
AASSLQS

SEQ ID NO: 212 - protein, 7 aa, Homo sapiens
AAASLQS

SEQ ID NO: 213 - protein, 9 aa, Homo sapiens
QQSYSSPIT

SEQ ID NO: 214 - protein, 9 aa, Homo sapiens
QQSYSAPIT

SEQ ID NO: 215 - protein, 10 aa, Homo sapiens
GFTFSSYAMN

SEQ ID NO: 216 - protein, 17 aa, Homo sapiens
TISGSGDNTYYADSVKG

SEQ ID NO: 217 - protein, 17 aa, Homo sapiens
TISGSGGNTYYADSVKG

SEQ ID NO: 218 - protein, 12 aa, Homo sapiens
KFVLMVYAMLDY

SEQ ID NO: 219 - protein, 11 aa, Homo sapiens
RASQRISNYLS

SEQ ID NO: 220 - protein, 16 aa, Homo sapiens
RSSQSLLHSNGYNFLN

SEQ ID NO: 221 - protein, 14 aa, Homo sapiens
TGTSSDVGNYNLVS

SEQ ID NO: 222 - protein, 14 aa, Homo sapiens
TGSSSNIGAGYDVH

SEQ ID NO: 223 - protein, 14 aa, Homo sapiens
TGSSSNIGAHYDVH

SEQ ID NO: 224 - protein, 13 aa, Homo sapiens
SGSNSNIGNNYVS

SEQ ID NO: 225 - protein, 11 aa, Homo sapiens
SGDKLGDKYAC

SEQ ID NO: 226 - protein, 12 aa, Homo sapiens
TLSSGYSSYEVD

SEQ ID NO: 227 - protein, 7 aa, Homo sapiens
LGSHRAS

SEQ ID NO: 228 - protein, 7 aa, Homo sapiens
EVSKRPS

SEQ ID NO: 229 - protein, 7 aa, Homo sapiens
GNSNRPS

SEQ ID NO: 230 - protein, 7 aa, Homo sapiens
GNTYRPS

SEQ ID NO: 231 - protein, 7 aa, Homo sapiens
SNNQRPS

SEQ ID NO: 232 - protein, 7 aa, Homo sapiens
DNNKRPS

SEQ ID NO: 233 - protein, 7 aa, Homo sapiens
QNTKWPL

SEQ ID NO: 234 - protein, 7 aa, Homo sapiens
VDTGGIV

SEQ ID NO: 235 - protein, 9 aa, Homo sapiens
QQSYSTPLI

SEQ ID NO: 236 - protein, 9 aa, Homo sapiens
MQVLQTPFT

SEQ ID NO: 237 - protein, 10 aa, Homo sapiens
CSYAGSSTLV

SEQ ID NO: 238 - protein, 11 aa, Homo sapiens
QSYDSSLSGSV

SEQ ID NO: 239 - protein, 11 aa, Homo sapiens
QSYDNSLSGVV

SEQ ID NO: 240 - protein, 11 aa, Homo sapiens
AVWDDSLNGWV

SEQ ID NO: 241 - protein, 11 aa, Homo sapiens
GTWDSSLSAVV

SEQ ID NO: 242 - protein, 9 aa, Homo sapiens
QAWDSSTVV

SEQ ID NO: 243 - protein, 18 aa, Homo sapiens
SDYHCGADHGSGTNFVVV

SEQ ID NO: 244 - protein, 10 aa, Homo sapiens
GYTFTSYGIS

SEQ ID NO: 245 - protein, 10 aa, Homo sapiens
GFTFSSYAMS

SEQ ID NO: 246 - protein, 10 aa, Homo sapiens
GFTFSSYGMH

SEQ ID NO: 247 - protein, 10 aa, Homo sapiens
GFTFSSYSMN

SEQ ID NO: 248 - protein, 12 aa, Homo sapiens
GGSISSGGYYWS

SEQ ID NO: 249 - protein, 12 aa, Homo sapiens
GGSISSSDYYWS

SEQ ID NO: 250 - protein, 10 aa, Homo sapiens
GGSFSAYYWN

SEQ ID NO: 251 - protein, 12 aa, Homo sapiens
GDSVSSNSAAWN

SEQ ID NO: 252 - protein, 17 aa, Homo sapiens
WISTYNGNTNYAQKVQG

SEQ ID NO: 253 - protein, 17 aa, Homo sapiens
TISGSGGRTYYADSVKG

SEQ ID NO: 254 - protein, 17 aa, Homo sapiens
VIWYDGSDKYYADSVKG

SEQ ID NO: 255 - protein, 17 aa, Homo sapiens
IIWYDGSNKYYADSVKG

SEQ ID NO: 256 - protein, 17 aa, Homo sapiens
SISSSSSYISYADSVKG

SEQ ID NO: 257 - protein, 16 aa, Homo sapiens
YIYNSGSTYYNPSLKS

SEQ ID NO: 258 - protein, 16 aa, Homo sapiens
YIYYSGSTYYNPSLKS

SEQ ID NO: 259 - protein, 16 aa, Homo sapiens
EINHSGRTDYNPSLKS

SEQ ID NO: 260 - protein, 18 aa, Homo sapiens
RTYYRSKWYKNYSVSVKS

SEQ ID NO: 261 - protein, 6 aa, Homo sapiens
GYTRDY

SEQ ID NO: 262 - protein, 8 aa, Homo sapiens
EVGSPFDY

SEQ ID NO: 263 - protein, 14 aa, Homo sapiens
ETGPLKLYYYGMDV

SEQ ID NO: 264 - protein, 13 aa, Homo sapiens
RGGLAARPGGMDV

SEQ ID NO: 265 - protein, 14 aa, Homo sapiens
DYDFWSAYYDAFDV

SEQ ID NO: 266 - protein, 11 aa, Homo sapiens
EDTAMVPYFDY

SEQ ID NO: 267 - protein, 12 aa, Homo sapiens
GGVTTYYYAMDV

SEQ ID NO: 268 - protein, 8 aa, Homo sapiens
GQLVPFDY

SEQ ID NO: 269 - protein, 9 aa, Homo sapiens
GGPTAAFDY

SEQ ID NO: 270 - protein, 109 aa, Homo sapiens
QSALTQPASVSGSPGQSITISCTGTSSDVGGYNSVSWYQQHPGKAPKLMIYEVSNRPSGVFNRFSGSKSGNTASLTISGLQAEDEADYYCNSYTSTSMVFGGGTKLTVL

SEQ ID NO: 271 - protein, 109 aa, Homo sapiens
QSALTQPASVFGSPGQSITISCTGTSSDVGAYNSVSWYQQHPGKAPKRMIYEVSNRPSGVSNRFSGSKSGNTASLTISGLQAEDEADYYCSSYTSTNMVFGGGTKLTVL

SEQ ID NO: 272 - protein, 109 aa, Homo sapiens; identical to SEQ ID NO: 31

SEQ ID NO: 273 - protein, 109 aa, Homo sapiens
QSVLTQPPSASGPPGQRVTIFCSGSSSNIGSNTVNWYQQLPGTAPKLLIYSNNRRPSGVPDRFSGSKSGTSASLAISGLQSEDEADYYCAAWDDSLNWVFGGGTKLTVL

SEQ ID NO: 274 - protein, 106 aa, Homo sapiens
SYELTQPPSVSVSPGQTASITCSGDKLGDKYACWYQQKPGQSPVLVIYQDSKRPSGIPERFSGSNSGNTATLTISGTQAMDEADYYCQAWDSSTVVFGGGTKLTVL

SEQ ID NO: 275 - protein, 106 aa, Homo sapiens; identical to SEQ ID NO: 44

SEQ ID NO: 276 - protein, 107 aa, Homo sapiens; identical to SEQ ID NO: 43

SEQ ID NO: 277 - protein, 107 aa, Homo sapiens
SYELIQPPSVSVSPGQTASITCSGDKLGDKYACWYQRKPGQSPILVIYQDTKRPSGIPERFSGSNSGNTATLTISGTQAMDEADYYCQAWDSSTAVVFGGGTKLTVL

SEQ ID NO: 278 - protein, 120 aa, Homo sapiens
QVQLQESGPGLVKPSETLSLTCTVSGGSISTYYWSWIRQPPGKGLEWIGYIYYSGSTNYNPSLKSRVTISVDTSKNQFSLKLSSVTAADTAVYYCARGSYSSGWFEFDYWGQGTLVTVSS

SEQ ID NO: 279 - protein, 12 aa, Homo sapiens
TLSSGYSSYEVD

SEQ ID NO: 280 - protein, 12 aa, Homo sapiens
VDTGGIVGSKGE

SEQ ID NO: 281 - protein, 13 aa, Homo sapiens
GADHGSGTNFVVV

SEQ ID NO: 282 - protein, 22 aa, Homo sapiens
QPVLTQPLFASASLGASVTLTC

SEQ ID NO: 283 - protein, 15 aa, Homo sapiens
WYQQRPGKGPRFVMR

SEQ ID NO: 284 - protein, 32 aa, Homo sapiens
GIPDRFSVLGSGLNRYLTIKNIQEEDESDYHC

SEQ ID NO: 285 - protein, 10 aa, Homo sapiens
FGGGTKLTVL

SEQ ID NO: 286 - protein, 108 aa, Homo sapiens
QSALTQPASVSGSPGQSITISCTGTSSDVGRYNSVSWYQHHPGKAPKVMIYEVSNRPSGVSTRFSGSKSGNTASLTISGLQAEDEADYYCSSYTSSSVVFGGGTKLTV

SEQ ID NO: 287 - protein, 108 aa, Homo sapiens
QSALTQPASVSGSPGQSITISCTGTSSDVGGYNSVSWYQQHPGKPPKLMIYEVSNRPSGVSIRFSGSKSGNTASLTISGLQAEDEADYFCSSYTSTSMVFGGGTKLTV

SEQ ID NO: 288 - protein, 108 aa, Homo sapiens
QSALTQPASVSGSPGQSITISCTGTNSDVGGYNSVSWYQQHPGKPPKLMIYEVSNRPSGISNRFSGSKSGNTASLTISGLQAEDEADYFCSSYTSTSMVFGGGTKLTV

SEQ ID NO: 289 - protein, 122 aa, Homo sapiens
QVHLVESGGGVVQPGRSLRLSCAASGFTFSSFGMHWVRQAPGKGLEWVALIWNDGSNKYYADSVKGRFTISRDNSKNTLYLQMNSLRAEDTAVYYCARAIAALYYYYGMDVWGHGTTVTVSS

SEQ ID NO: 290 - protein, 122 aa, Homo sapiens
QVQLVESGGGVVQPGRSLRLSCAASGFTFSSYGMHWVRQAPGKGLECVAIIWYDGSNKYYADSVKGRFTISRDNSKNTLYLQMNSLRAEDTAVYYCARRGGLAARPGGMDVWGQGTTVTVSS

SEQ ID NO: 291 - protein, 121 aa, Homo sapiens
QVQLVESGGGVVQPGRSLRLSCAASGFTFSSFGMHWVRQAPGKGLEWVALIWNDGSNKYYADSVKGRFTISRDNSKNTLYLQMNSLRAEDTAVYYCARAIAALYYYYGMDVWGQGTTVTVS

SEQ ID NO: 292 - protein, 119 aa, Homo sapiens
QVQLVESGGGVVQPGRSLRLSCAASGFTFSSYGMHWVRQAPGKGLEWVAIIWYDGSNKYYADSVKGRFTISRDNSKNTLYLQMNSLRAEDTAVYYCARRGGLPGGMDVWGQGTTVTVSS

SEQ ID NO: 293 - DNA, 327 bp, Homo sapiens
cagtctgccctgactcagcctgcctccgtgtctgggtctcctggacagtcgatcaccatctcctgcactggaaccagcagtgacgttggtggttataactctgtctcctggtaccaacagcacccaggcaaagcccccaaactcatgatttatgaggtcagtaatcggccctcaggggtttctaatcgcttctctggctccaagtctggcaacacggcctccctgaccatctctgggctccaggctgaggacgaggctgattattactgcaactcatatacaagcaccagcatggtattcggcggagggaccaagctgaccgtccta

SEQ ID NO: 294 - DNA, 327 bp, Homo sapiens
cagtctgccctgactcagcctgcctccgtgtctgggtctcctggacagtcgatcaccatctcctgcactggaaccagcagtgacgttggtggttataactctgtctcctggtaccaacagcacccaggcaaaccccccaaactcatgatttatgaggtcagtaatcggccctcaggggtttctaatcgcttctctggctccaagtctggcaacacggcctccctgaccatctctgggctccaggctgaggacgaggctgattatttctgcagctcatatacaagcaccagcatggtcttcggcggagggaccaagctgaccgtccta

SEQ ID NO: 295 - DNA, 318 bp, Homo sapiens
tcctatgagctgactcagccaccctcagtgtccgtgtccccaggacagacagccagaatcacctgctctggagataaattgggggataaatatgcttgctggtatcagcagaagccaggccagtcccctgtgctggtcatctatcaaaataccaagtggcccttagggatccctgagcgattctctggctccaagtctgggaacacagtcactctgaccatcagcgggacccaggctatggatgaggctgactattactgtcaggcgtgggacagcagcactgtggtattcggcggagggaccaagctgaccgtccta

SEQ ID NO: 296 - DNA, 327 bp, Homo sapiens; identical to SEQ ID NO: 95

SEQ ID NO: 297 - protein, 215 aa, Homo sapiens
ESALTQPASVSGSPGQSITISCTGTSSDVGGYNSVSWYQQHPGKAPKLMIYEVSNRPSGVSNRFSGSKSGNTASLTISGLQAEDEADYYCNSYTSTSMVFGGGTKLTVLGQPKAAPSVTLFPPSSEELQANKATLVCLISDFYPGAVTVAWKADSSPVKAGVETTTPSKQSNNKYAASSYLSLTPEQWKSHRSYSCQVTHEGSTVEKTVAPTECS

SEQ ID NO: 298 - protein, 230 aa, Homo sapiens
EVQLVQSGAEVKKPGASVKVSCKASGYTLTSYGISWVRQAPGQGLEWMGWVSFYNGNTNYAQKLQGRGTMTTDPSTSTAYMELRSLRSDDTAVYYCARGYGMDVWGQGTTVTVSSASTKGPSVFPLAPSSKSTSGGTAALGCLVKDYFPEPVTVSWNSGALTSGVHTFPAVLQSSGLYSLSSVVTVPSSSLGTQTYICNVNHKPSNTKVDKKVEPKSCAADEVDHHHHHH

SEQ ID NO: 299 - protein, 217 aa, Homo sapiens
ESVLTQPPSVSGAPGQRVTISCTGSSSNIGAGYDVHWYQQLPGTAPKLLISGNSNRPSGVPDRFSGSKSGTSASLAITGLQAEDEADYYCQSYDSSLSGSVFGGGTKLTVLGQPKAAPSVTLFPPSSEELQANKATLVCLISDFYPGAVTVAWKADSSPVKAGVETTTPSKQSNNKYAASSYLSLTPEQWKSHRSYSCQVTHEGSTVEKTVAPTECS

SEQ ID NO: 300 - protein, 238 aa, Homo sapiens
EVQLVESGGGLVKPGGSLRLSCAASGFTFSSYSMNWVRQAPGKGLEWVSSISSSSSYISYADSVKGRFTISRDNAKNSLYLQMNSLRAEDTAVYFCARDYDFWSAYYDAFDVWGQGTMVTVSSASTKGPSVFPLAPSSKSTSGGTAALGCLVKDYFPEPVTVSWNSGALTSGVHTFPAVLQSSGLYSLSSVVTVPSSSLGTQTYICNVNHKPSNTKVDKKVEPKSCAADEVDHHHHHH

SEQ ID NO: 301 - protein, 218 aa, Homo sapiens
ALQSVLTQPPSASGTPGQRVTISCSGSSSNIGSNTVNWYQQLPGTAPKLLIYSNNQRPSGVPDRFSGSKSGTSASLAISGLQSEDEADYYCAVWDDSLNGWVFGGGTKLTVLGQPKAAPSVTLFPPSSEELQANKATLVCLISDFYPGAVTVAWKADSSPVKAGVETTTPSKQSNNKYAASSYLSLTPEQWKSHRSYSCQVTHEGSTVEKTVAPTECS

SEQ ID NO: 302 - protein, 231 aa, Homo sapiens
QVQLQQWGAGLLKPSETLSLTCAVYGGSFSAYYWNWIRQPPGKGLEWIGEINHSGRTDYNPSLKSRVTISVDTSKKQFSLKLNSVTAADTAVYYCARGQLVPFDYWGQGTLVTVSSASTKGPSVFPLAPSSKSTSGGTAALGCLVKDYFPEPVTVSWNSGALTSGVHTFPAVLQSSGLYSHSSVVTVPSSSLGTQTYICNVNHKPSNTKVDKKVEPKSCAADEVDHHHHHH

SEQ ID NO: 303 - protein, 680 aa, Homo sapiens
QEDEDGDYEELVLALRSEEDGLAEAPEHGTTATFHRCAKDPWRLPGTYVVVLKEETHLSQSERTARRLQAQAARRGYLTKILHVFHGLLPGFLVKMSGDLLELALKLPHVDYIEEDSSVFAQSIPWNLERITPPRYRADEYQPPDGGSLVEVYLLDTSIQSDHREIEGRVMVTDFENVPEEDGTRFHRQASKCDSHGTHLAGVVSGRDAGVAKGASMRSLRVLNCQGKGTVSGTLIGLEFIRKSQLVQPVGPLVVLLPLAGGYSRVLNAACQRLARAGVVLVTAAGNFRDDACLYSPASAPEVITVGATNAQDQPVTLGTLGTNFGRCVDLFAPGEDIIGASSDCSTCFVSQSGTSQAAAHVAGIAAMMLSAEPELTLAELRQRLIHFSAKDVINEAWFPEDQRVLTPNLVAALPPSTHGAGWQLFCRTVWSAHSGPTRMATAIARCAPDEELLSCSSFSRSGKRRGERMEAQGGKLVCRAHNAFGGEGVYAIARCCLLPQANCSVHTAPPAEASMGTRVHCHQQGHVLTGCSSHWEVEDLGTHKPPVLRPRGQPNQCVGHREASIHASCCHAPGLECKVKEHGIPAPQEQVTVACEEGWTLTGCSALPGTSHVLGAYAVDNTCVVRSRDVSTTGSTSEEAVTAVAICCRSRHLAQASQELQGSSDYKDDDKHHHHHHHH

SEQ ID NO: 304 - protein, 680 aa, Homo sapiens
RRRRRRRRRRRRLRRRRRRRRRRRRRRHRRRRRFRRCRRRPWRRPGRYVVVLRRRRRRSRSRETAEELQRRAREEGRRTKIRRRFRGLLPGFLVRMRRRLRRLARRLPRVRYIEEDSSVFRQRIPRNRREIRPPRYRARRRRPPRGGRRVEVYLLDTRIRRRHEEIRGRVRRRRFRRRPRRRRREREERRRRCDRRGTHLAGVVSGERAGVARRARMRSLEVLNCRGRGRVSGTLIGLERIERRRRRRPRRPLVVLLPLAGRYSEVLNRACRRLAERGVVLVTAAGNFEDDACRYSPARAPEVITVGATNRRRRPVRRGRRGTNFGRCVDLFAPGRRIIGASSRCSRCRRRRSGTSQAAAHVAGIAARMLRRRPRLRRARLRQELRRRSRRRRIRRRRFPRRRERLTPRLVARLPPRRRRRGRRLFCRTVWSRRSGPRERARAIAECAPREELLSCSSFSRSGKRRGERMERQGGKLVCRAHNARRGRGVYAIARCCLLPQARCSVHRAPPARRRRGTEVRCRRRGHVLTGCSSHWRRRDRGTRKPPRLRPEGRPRQCVGHREASIHASCCHAPGLECRRRRRRIPAPRERVTVRCRRGWTLTGCSALPGTSHVLGAYARDNTCVVRSEDRRRRRRRRRERVTAVAICCESEHLAQASQELQGSSDYKDDDKHHHHHHHH

SEQ ID NO: 305 - protein, 14 aa, Homo sapiens
TGTSSDVGGYNSVS

SEQ ID NO: 306 - protein, 7 aa, Homo sapiens
EVSNRPS

SEQ ID NO: 307 - protein, 9 aa, Homo sapiens
SSYTSTSMV

SEQ ID NO: 308 - protein, 5 aa, Homo sapiens
SYGIS

SEQ ID NO: 309 - protein, 17 aa, Homo sapiens
WISAYNGNTNYAQKVQG

SEQ ID NO: 310 - protein, 6 aa, Homo sapiens
GYGMDV

SEQ ID NO: 311 - protein, 14 aa, Homo sapiens
TGTSSDVGRYNSVS

SEQ ID NO: 312 - protein, 7 aa, Homo sapiens
EVSNRPS

SEQ ID NO: 313 - protein, 9 aa, Homo sapiens
SSYTSSSVV

SEQ ID NO: 314 - protein, 17 aa, Homo sapiens
WISAYNGNTNYAEKLQG

SEQ ID NO: 315 - protein, 6 aa, Homo sapiens
GYVMDV

SEQ ID NO: 316 - protein, 14 aa, Homo sapiens
TGTSSDVGAYNSVS

SEQ ID NO: 317 - protein, 9 aa, Homo sapiens
SSYTSTNMV

SEQ ID NO: 318 - protein, 17 aa, Homo sapiens
WVSAYNGNTNYAQKFQG

SEQ ID NO: 319 - protein, 9 aa, Homo sapiens
NSYTSTSMV

SEQ ID NO: 320 - protein, 17 aa, Homo sapiens
WVSFYNGNTNYAQKLQG

SEQ ID NO: 321 - protein, 7 aa, Homo sapiens
EVTNRPS

SEQ ID NO: 322 - protein, 14 aa, Homo sapiens
TGTNSDVGGYNSVS

SEQ ID NO: 323 - protein, 17 aa, Homo sapiens
WISVYNGNTNYAQKVQG

SEQ ID NO: 324 - protein, 17 aa, Homo sapiens
WISFYNGNTNYAQKVQG

SEQ ID NO: 325 - protein, 13 aa, Homo sapiens
SGSSSNIGNNFVS

SEQ ID NO: 326 - protein, 7 aa, Homo sapiens
DYNKRPS

SEQ ID NO: 327 - protein, 11 aa, Homo sapiens
GTWDSSLSGYV

SEQ ID NO: 328 - protein, 5 aa, Homo sapiens
SFGMH

SEQ ID NO: 329 - protein, 17 aa, Homo sapiens
LIWNDGSNKYYADSVKG

SEQ ID NO: 330 - protein, 13 aa, Homo sapiens
AIAALYYYYGMDV

SEQ ID NO: 331 - protein, 7 aa, Homo sapiens
DSNKRPS

SEQ ID NO: 332 - protein, 11 aa, Homo sapiens
GTWDSSLSAYV

SEQ ID NO: 333 - protein, 5 aa, Homo sapiens
SYGMH

SEQ ID NO: 334 - protein, 17 aa, Homo sapiens
LIWHDGSNTYYVDSVKG

SEQ ID NO: 335 - protein, 13 aa, Homo sapiens
GIAVAYYYYGMDV

SEQ ID NO: 336 - protein, 17 aa, Homo sapiens
LIWSDGSDEYYADSVKG

SEQ ID NO: 337 - protein, 11 aa, Homo sapiens
GTWDSSLSSYV

SEQ ID NO: 338 - protein, 17 aa, Homo sapiens
LIWSDGSDKYYADSVKG

SEQ ID NO: 339 - protein, 13 aa, Homo sapiens
SGSSSNIGSKTVN

SEQ ID NO: 340 - protein, 7 aa, Homo sapiens
SNNRRPS

SEQ ID NO: 341 - protein, 10 aa, Homo sapiens
AAWDDSLNWV

SEQ ID NO: 342 - protein, 4 aa, Homo sapiens
YWMS

SEQ ID NO: 343 - protein, 17 aa, Homo sapiens
NIKQDGSEKYYVDSVKG

SEQ ID NO: 344 - protein, 10 aa, Homo sapiens
ESNWGFAFDI

SEQ ID NO: 345 - protein, 13 aa, Homo sapiens
SGSSSNIGSNTVN

SEQ ID NO: 346 - protein, 5 aa, Homo sapiens
RYWMS

SEQ ID NO: 347 - protein, 17 aa, Homo sapiens
NIKHDGSEKYYVDSVKG

SEQ ID NO: 348 - protein, 10 aa, Homo sapiens
ESNWGFAFDV

SEQ ID NO: 349 - protein, 7 aa, Homo sapiens
RNNQRPL

SEQ ID NO: 350 - protein, 5 aa, Homo sapiens
SYWMS

SEQ ID NO: 351 - protein, 5 aa, Homo sapiens
NFWMS

SEQ ID NO: 352 - protein, 10 aa, Homo sapiens
RASQSISYLN

SEQ ID NO: 353 - protein, 6 aa, Homo sapiens
AASLQS

SEQ ID NO: 354 - protein, 8 aa, Homo sapiens
QQSYSPIT

SEQ ID NO: 355 - protein, 11 aa, Homo sapiens
RASQSISIYLN

SEQ ID NO: 356 - protein, 7 aa, Homo sapiens
AAASLQS

SEQ ID NO: 357 - protein, 9 aa, Homo sapiens
QQSYSAPIT

SEQ ID NO: 358 - protein, 11 aa, Homo sapiens
RASQSISSYLN

SEQ ID NO: 359 - protein, 7 aa, Homo sapiens
AASSLQS

SEQ ID NO: 360 - protein, 9 aa, Homo sapiens
QQSYSSPIT

SEQ ID NO: 361 - protein, 5 aa, Homo sapiens
SYAMN

SEQ ID NO: 362 - protein, 16 aa, Homo sapiens
TISGSGNTYYADSVKG

SEQ ID NO: 363 - protein, 12 aa, Homo sapiens
KFVLMVYAMLDY

SEQ ID NO: 364 - protein, 17 aa, Homo sapiens
TISGSGGNTYYADSVKG

SEQ ID NO: 365 - protein, 17 aa, Homo sapiens
TISGSGDNTYYADSVKG

SEQ ID NO: 366 - protein, 10 aa, Homo sapiens
GYSLTSYGIS

SEQ ID NO: 367 - protein, 10 aa, Homo sapiens
GYALTSYGIS

SEQ ID NO: 368 - protein, 10 aa, Homo sapiens
GYTLTSYGIS

SEQ ID NO: 369 - protein, 10 aa, Homo sapiens
GYSFTSYGIS

SEQ ID NO: 370 - protein, 10 aa, Homo sapiens
GYTFPSYGIS

SEQ ID NO: 371 - protein, 10 aa, Homo sapiens
GFTFSSYWMS

SEQ ID NO: 372 - protein, 10 aa, Homo sapiens
GFTFSRYWMS

SEQ ID NO: 373 - protein, 10 aa, Homo sapiens
GLTFSNFWMS

SEQ ID NO: 374 - protein, 10 aa, Homo sapiens
GFTFSSYAMN

SEQ ID NO: 375 - protein, 10 aa, Homo sapiens
GFTFNSFGMH

SEQ ID NO: 376 - protein, 10 aa, Homo sapiens
GFTFRSYGMH

SEQ ID NO: 377 - protein, 16 aa, Homo sapiens
NIKQDGSEKYVDSVKG

SEQ ID NO: 378 - protein, 16 aa, Homo sapiens
NIKHDGSEKYVDSVKG

SEQ ID NO: 379 - protein, 16 aa, Homo sapiens
TISGSGDNTYADSVKG

SEQ ID NO: 380 - protein, 16 aa, Homo sapiens
TISGSGGNTYADSVKG

SEQ ID NO: 381 - protein, 16 aa, Homo sapiens
LIWNDGSNKYADSVKG

SEQ ID NO: 382 - protein, 16 aa, Homo sapiens
LIWSDGSDEYADSVKG

SEQ ID NO: 383 - protein, 16 aa, Homo sapiens
LIWSDGSDKYADSVKG

SEQ ID NO: 384 - protein, 16 aa, Homo sapiens
LIWHDGSNTYVDSVKG

SEQ ID NO: 385 - protein, 10 aa, Homo sapiens
ESNWGFAFDI

SEQ ID NO: 386 - protein, 10 aa, Homo sapiens
ESNWGFAFDV

SEQ ID NO: 387 - protein, 6 aa, Homo sapiens
GYVMDV

SEQ ID NO: 388 - protein, 11 aa, Homo sapiens
RASQSISIYLN

SEQ ID NO: 389 - protein, 14 aa, Homo sapiens
TGTNSDVGGYNSVS

SEQ ID NO: 390 - protein, 14 aa, Homo sapiens
TGTSSDVGAYNSVS

SEQ ID NO: 391 - protein, 14 aa, Homo sapiens
TGTSSDVGRYNSVS

SEQ ID NO: 392 - protein, 7 aa, Homo sapiens
RNNQRPL

SEQ ID NO: 393 - protein, 7 aa, Homo sapiens
AAASLQS

SEQ ID NO: 394 - protein, 9 aa, Homo sapiens
QQSYSAPIT

SEQ ID NO: 395 - protein, 9 aa, Homo sapiens
NSYTSTSMV

SEQ ID NO: 396 - protein, 9 aa, Homo sapiens
SSYTSSSVV

SEQ ID NO: 397 - protein, 10 aa, Homo sapiens
AAWDDSLNWV

SEQ ID NO: 398 - protein, 11 aa, Homo sapiens
GTWDSSLSSYV

SEQ ID NO: 399 - protein, 11 aa, Homo sapiens
GTWDSSLSAYV

SEQ ID NO: 400 - protein, 116 aa, Homo sapiens
QVQLQESGPGLVKPSETLSLTCTVSGGSISSYYWSWIRQPPGKGLEWIGYIYYSGSTNYNPSLKSRVTISVDTSKNQFSLKLSSVTAADTAVYYCARYSSGWFDYWGQGTLVTVSS

SEQ ID NO: 401 - protein, 118 aa, Homo sapiens
EVQLVESGGGLVQPGGSLRLSCVVSGFTFSSYWMSWVRQAPGKGLEWVANIKQDGSEKYYVDSVKGRFTISRDNAKNSLYLQMNSLRAEDTAVYYCARESNWGFAFDIWGQGTMVTVS

SEQ ID NO: 402 - protein, 115 aa, Homo sapiens
EVQLVESGGGLVQPGGSLRLSCAASGFTFSSYWMSWVRQAPGKGLEWVANIKQDGSEKYYVDSVKGRFTISRDNAKNSLYLQMNSLRAEDTAVYYCARNWGAFDIWGQGTMVTVS

SEQ ID NO: 403 - protein, 6 aa, Homo sapiens
ENLYFQ

SEQ ID NO: 404 - protein, 14 aa, Homo sapiens
  VARIANT 1: Xaa= D, A, R or no amino acid
  VARIANT 2: Xaa=Y, I, G or no amino acid
  VARIANT 3: Xaa=D, A, G or no amino acid
  VARIANT 4: Xaa=F, A, L or no amino acid
  VARIANT 5: Xaa=W, L, A or no amino acid
  VARIANT 6: Xaa=S, Y, A or no amino acid
  VARIANT (7)...(7): Xaa=A, Y, R or no amino acid
  VARIANT (8)...(8): Xaa=Y,  P or no amino acid
  VARIANT (9)...(9): Xaa=Y, G or no amino acid
  VARIANT (10)...(10): Xaa=D, G or no amino acid
  VARIANT (11)...(11): Xaa=A, M or no amino acid
  VARIANT (12)...(12): Xaa=F,D  or no amino acid
  VARIANT (13)...(13): Xaa=D, V or no amino acid
  VARIANT (14)...(14): Xaa=V or no amino acid
XXXXXXXXXXXXXX

SEQ ID NO: 405 - protein, 11 aa, Homo sapiens
  VARIANT 1: Xaa=Q or G
  VARIANT 2: Xaa=S, T, A or no amino acid
  VARIANT 3: Xaa=Y, W or no amino acid
  VARIANT 4: Xaa=D or no amino acid
  VARIANT 5: Xaa=S or no amino acid
  VARIANT 6: Xaa=S or no amino acid
  VARIANT (7)...(7): Xaa=L, T or no amino acid
  VARIANT (8)...(8): Xaa=A, S or no amino acid
  VARIANT (9)...(9): Xaa=G, A, V or no amino acid
  VARIANT (10)...(10): Xaa=S, Y, V or no amino acid
  VARIANT (11)...(11): Xaa=V or no amino acid
XXXXXXXXXXX

SEQ ID NO: 406 - protein, 10 aa, Homo sapiens
  VARIANT 1: Xaa=G
  VARIANT 2: Xaa=Y, F or G
  VARIANT 3: Xaa=T or S
  VARIANT 4: Xaa=L or F
  VARIANT 5: Xaa=T, S or N
  VARIANT 6: Xaa=S or A
  VARIANT (7)...(7): Xaa=Y or F
  VARIANT (8)...(8): Xaa=G, S or Y
  VARIANT (9)...(9): Xaa=I, M or W
  VARIANT (10)...(10): Xaa=S, N or H
XXXXXXXXXX

SEQ ID NO: 407 - protein, 14 aa, Homo sapiens
  VARIANT 1: Xaa=T or no amino acid
  VARIANT 2: Xaa=G or S
  VARIANT 3: Xaa=S, T or G
  VARIANT 4: Xaa=S
  VARIANT 5: Xaa=S
  VARIANT 6: Xaa=N, D or S
  VARIANT (7)...(7): Xaa=I, V or N
  VARIANT (8)...(8): Xaa=G or I
  VARIANT (9)...(9): Xaa=A or G
  VARIANT (10)...(10): Xaa=G, Y, S or N
  VARIANT (11)...(11): Xaa=Y or N
  VARIANT (12)...(12): Xaa=D, S, T or F
  VARIANT (13)...(13): Xaa=V
  VARIANT (14)...(14): Xaa=S, N or H
XXXXXXXXXXXXXX

SEQ ID NO: 408 - protein, 17 aa, Homo sapiens
  VARIANT 1: Xaa=W, S, L or no amino acid
  VARIANT 2: Xaa=V, I or E
  VARIANT 3: Xaa=S, W or I
  VARIANT 4: Xaa=F, S or N
  VARIANT 5: Xaa=Y, S, D or H
  VARIANT 6: Xaa=N, S or G
  VARIANT (7)...(7): Xaa=S or G
  VARIANT (8)...(8): Xaa=N, Y, D or R
  VARIANT (9)...(9): Xaa=T, I or E
  VARIANT (10)...(10): Xaa=N, S, Y or D
  VARIANT (11)...(11): Xaa=Y
  VARIANT (12)...(12): Xaa=A and N
  VARIANT (13)...(13): Xaa=Q, D or P
  VARIANT (14)...(14): Xaa=K or S
  VARIANT (15)...(15): Xaa=L or V
  VARIANT (16)...(16): Xaa=Q or K
  VARIANT (17)...(17): Xaa=G or S
XXXXXXXXXXXXXXXXX

SEQ ID NO: 409 - protein, 7 aa, Homo sapiens
  VARIANT 1: Xaa=G, E, S or D
  VARIANT 2: Xaa=N, V or Y
  VARIANT 3: Xaa=S or N
  VARIANT 4: Xaa=N, Q or K
  VARIANT 5: Xaa=R
  VARIANT 6: Xaa=P
  VARIANT (7)...(7): Xaa=S
XXXXXXX

SEQ ID NO: 410 - protein, 14 aa, Homo sapiens
  VARIANT 1: Xaa=D or no amino acid
  VARIANT 2: Xaa=Y, A or no amino acid
  VARIANT 3: Xaa=D, I or no amino acid
  VARIANT 4: Xaa=F, A or no amino acid
  VARIANT 5: Xaa=W, A or no amino acid
  VARIANT 6: Xaa=S, L or no amino acid
  VARIANT (7)...(7): Xaa=A, Y, G or no amino acid
  VARIANT (8)...(8): Xaa=Y, Q or no amino acid
  VARIANT (9)...(9): Xaa=G, Y or L
  VARIANT (10)...(10): Xaa=Y, D or V
  VARIANT (11)...(11): Xaa=G, A or P
  VARIANT (12)...(12): Xaa=M or F
  VARIANT (13)...(13): Xaa=D
  VARIANT (14)...(14): Xaa=V or Y
XXXXXXXXXXXXXX

SEQ ID NO: 411 - protein, 11 aa, Homo sapiens
  VARIANT 1: Xaa=Q, A, G or no amino acid
  VARIANT 2: Xaa=S, V, T or no amino acid
  VARIANT 3: Xaa=Y, N or W
  VARIANT 4: Xaa=S or D
  VARIANT 5: Xaa=S, Y or D
  VARIANT 6: Xaa=S or T
  VARIANT (7)...(7): Xaa=L or S
  VARIANT (8)...(8): Xaa=S, T or N
  VARIANT (9)...(9): Xaa=G, S or A
  VARIANT (10)...(10): Xaa=S, M, W or Y
  VARIANT (11)...(11): Xaa=V
XXXXXXXXXXX

SEQ ID NO: 412 - protein, 10 aa, Homo sapiens
  VARIANT 1: Xaa=G, P or A
  VARIANT 2: Xaa=Y, W, F, T or S
  VARIANT 3: Xaa=T, P, S, A, C, V, L or I
  VARIANT 4: Xaa=L, F, I, V, M, A or Y
  VARIANT 5: Xaa=T, P, S or A
  VARIANT 6: Xaa=S, T, A or C
  VARIANT (7)...(7): Xaa=Y, W, F, T or S
  VARIANT (8)...(8): Xaa=G, P or A
  VARIANT (9)...(9): Xaa=I, L, V, M, A or F
  VARIANT (10)...(10): Xaa=S, T, A or C
XXXXXXXXXX

SEQ ID NO: 413 - protein, 14 aa, Homo sapiens
  VARIANT 1: Xaa=T or S
  VARIANT 2: Xaa=G, P or A
  VARIANT 3: Xaa=T or S
  VARIANT 4: Xaa=S, N, T, A, C or Q
  VARIANT 5: Xaa=S, T, A or C
  VARIANT 6: Xaa=D or E
  VARIANT (7)...(7): Xaa=V, I, M, L, F or A
  VARIANT (8)...(8): Xaa=G, P or A
  VARIANT (9)...(9): Xaa=G, A, R, P, V, L, I, K, Q or N
  VARIANT (10)...(10): Xaa=Y, W, F, T or S
  VARIANT (11)...(11): Xaa=N or Q
  VARIANT (12)...(12): Xaa=Y, S, W, F, T, S, T, A or C
  VARIANT (13)...(13): Xaa=V, I, M, L, F, or A
  VARIANT (14)...(14): Xaa=S, T, A or C
XXXXXXXXXXXXXX

SEQ ID NO: 414 - protein, 17 aa, Homo sapiens
  VARIANT 1: Xaa=W, Y or F
  VARIANT 2: Xaa=V, I, M, L, F or A
  VARIANT 3: Xaa=S, T, A or C
  VARIANT 4: Xaa=A, F, V, L, I, Y or M
  VARIANT 5: Xaa=Y, W, F, T or S
  VARIANT 6: Xaa=N or Q
  VARIANT (7)...(7): Xaa=G, P or A
  VARIANT (8)...(8): Xaa=N or Q
  VARIANT (9)...(9): Xaa=T or S
  VARIANT (10)...(10): Xaa=N or Q
  VARIANT (11)...(11): Xaa=Y, W, F, T or S
  VARIANT (12)...(12): Xaa=A, V, L or I
  VARIANT (13)...(13): Xaa=Q, E, N or D
  VARIANT (14)...(14): Xaa=K, R, Q or N
  VARIANT (15)...(15): Xaa=L, F, V, I, M, A or Y
  VARIANT (16)...(16): Xaa=Q or N
  VARIANT (17)...(17): Xaa=G, P or A
XXXXXXXXXXXXXXXXX

SEQ ID NO: 415 - protein, 7 aa, Homo sapiens
  VARIANT 1: Xaa=E or D
  VARIANT 2: Xaa=V, I, M, L, F or A
  VARIANT 3: Xaa=S, T, A or C
  VARIANT 4: Xaa=N or Q
  VARIANT 5: Xaa=R, K, Q or N
  VARIANT 6: Xaa=P or A
  VARIANT (7)...(7): Xaa=S, T, A or C
XXXXXXX

SEQ ID NO: 416 - protein, 6 aa, Homo sapiens
  VARIANT 1: Xaa=G, P, A or no amino acid
  VARIANT 2: Xaa=Y, W, F, T or S
  VARIANT 3: Xaa=G, V, P, A, I, M, L or F
  VARIANT 4: Xaa=M, L, F or I
  VARIANT 5: Xaa=D or E
  VARIANT 6: Xaa=V, I, M, L, F or A
XXXXXX

SEQ ID NO: 417 - protein, 9 aa, Homo sapiens
  VARIANT 1: Xaa=S, N, T, A, C or Q
  VARIANT 2: Xaa=S, T, A or C
  VARIANT 3: Xaa=Y, W, F, T or S
  VARIANT 4: Xaa=T or S
  VARIANT 5: Xaa=S, T, A or C
  VARIANT 6: Xaa=S, T, A or C
  VARIANT (7)...(7): Xaa=N, S, Q, T, A or C
  VARIANT (8)...(8): Xaa=M, V, L, F, I or A
  VARIANT (9)...(9): Xaa=V, I, M, L, F or A
XXXXXXXXX

SEQ ID NO: 418 - DNA, 363 bp, Homo sapiens
caggtgcaggtggtgcagtctggggctgaggtgaagaagcctggggcctcagtgaaggtctcctgcaaggcttctggatacaccttcaccggctactatatacactgggtgcgacaggcccctggacaagggcttgagtggatgggatggatcaaccctcacagtggtggcgcaaactatgcacagaagtttcagggcagggtcaccatgaccagggacacgtccatcagcacagcctacatggagctgagcaggctgagatctgacgacacggccgtgtattactgtgcgagaggcaactggaactacgactactacggtatggacgtctggggccaagggaccacggtcaccgtctcctca

SEQ ID NO: 419 - protein, 121 aa, Homo sapiens
QVQVVQSGAEVKKPGASVKVSCKASGYTFTGYYIHWVRQAPGQGLEWMGWINPHSGGANYAQKFQGRVTMTRDTSISTAYMELSRLRSDDTAVYYCARGNWNYDYYGMDVWGQGTTVTVSS

SEQ ID NO: 420 - DNA, 321 bp, Homo sapiens
gacatccagatgacccagtctccatcctccctgtctgcatctgtaggagacagagtcaccatcacttgccgggcgagtcaggacattagcaattatttagcctggtatcagcagaaaccagggaaagttcctaagctcctgatctatgctgcatccactttgcaatcaggggtcccatctcggttcagtggcagtggatctgggacagatttcactctcaccatcagcagcctacagcctgaagatgttgcaacttatttctgtcaaaggtatcagattgccccattcactttcggccctgggaccaaggtggatatcaaa

SEQ ID NO: 421 - protein, 107 aa, Homo sapiens
DIQMTQSPSSLSASVGDRVTITCRASQDISNYLAWYQQKPGKVPKLLIYAASTLQSGVPSRFSGSGSGTDFTLTISSLQPEDVATYFCQRYQIAPFTFGPGTKVDIK

SEQ ID NO: 422 - DNA, 366 bp, Homo sapiens
caggtgcagctggtggagtctgggggaggcgtggtccagcctgggaggtccctgagactctcctgtgcagcgtctggattcaccttcagtagctatggcatgcactgggtccgccaggctccaggcaaggggctggagtgggtggcagttatctggtatgatggaagtactaaatactatgcagactccgtgaagggccgatccaccatctccagagacaattccaagaacacgctgtatctgcaaatgaacagcctgagagccgaggacacggctgtgtattactgtgcgaggtcagtggctggttaccactactactacggtatggacgtctggggccaagggaccacggtcaccgtctcctca

SEQ ID NO: 423 - protein, 122 aa, Homo sapiens
QVQLVESGGGVVQPGRSLRLSCAASGFTFSSYGMHWVRQAPGKGLEWVAVIWYDGSTKYYADSVKGRSTISRDNSKNTLYLQMNSLRAEDTAVYYCARSVAGYHYYYGMDVWGQGTTVTVSS

SEQ ID NO: 424 - DNA, 324 bp, Homo sapiens
tcttctgagctgactcaggaccctgctgtgtctgtggccttgggacagacagtcaggatcacatgccaaggagacagcctcagaggctattatgcaacctggtaccagcagaagccaagacaggcccctgtacttgtcatctatggtaaaaactaccggccctcagggatcccagaccgattctctggctccacctcaggaaacacagcttccttgaccatcactggggctcaggcggaagatgaggctgactattactgtaactcccgggacagcattggtaaccatctggtgttcggcggagggaccaagctgaccgtccta

SEQ ID NO: 425 - protein, 108 aa, Homo sapiens
SSELTQDPAVSVALGQTVRITCQGDSLRGYYATWYQQKPRQAPVLVIYGKNYRPSGIPDRFSGSTSGNTASLTITGAQAEDEADYYCNSRDSIGNHLVFGGGTKLTVL

SEQ ID NO: 426 - DNA, 366 bp, Homo sapiens
caggtgcagctggtggagtctgggggaggcgtggtccagcctgggaggtccctgagactctcctgtgcagcgtctggattcaccttcagtagctatggcttgcactgggtccgccaggctccaggcaaggggctggagtgggtggcagttatatggttagatggaagtaataaatactatgcagactccgtgaagggccgatccaccatctccagagacaattccaagaacacgctgtatctgcaaatgaacagcctgagagccgaggacacggctgtgtattactgtgcgaggtcagtggctggttaccactactactacggtatggacgtctggggccaagggaccacggtcaccgtctcctca

SEQ ID NO: 427 - protein, 122 aa, Homo sapiens
QVQLVESGGGVVQPGRSLRLSCAASGFTFSSYGLHWVRQAPGKGLEWVAVIWLDGSNKYYADSVKGRSTISRDNSKNTLYLQMNSLRAEDTAVYYCARSVAGYHYYYGMDVWGQGTTVTVSS

SEQ ID NO: 428 - DNA, 324 bp, Homo sapiens
tcttctgagctgactcaggaccctgctgtgtctgtggccttgggacagacagtcaggatcacatgccaaggagacagcctcagaagttattatggaagctggtaccagcagaagccaagacaggcccctgtacttgtcatctttggtaaaaacaaccggccctcagggatcccagaccgattctctggctccacctcaggaaacacagcttccttgaccatcactggggctcaggcggaagatgaggctgactattactgtaactcacgggacatcattggtgaccatctgctgttcggcggagggaccaagctgaccgtccta

SEQ ID NO: 429 - protein, 108 aa, Homo sapiens
SSELTQDPAVSVALGQTVRITCQGDSLRSYYGSWYQQKPRQAPVLVIFGKNNRPSGIPDRFSGSTSGNTASLTITGAQAEDEADYYCNSRDIIGDHLLFGGGTKLTVL

SEQ ID NO: 430 - DNA, 366 bp, Homo sapiens
caggtgcagctggtggagtctgggggaggcgtggtccagtctgggaggtccctgagactctcctgtgcagcgtctggattcaccttcaggaactatggcatgcactgggtccgccaggctccaggcaaggggctggagtgggtggcagttatatggtttgatggaagtaataaatactatgcagactccgtgaagggccgatccaccatctccagagacaattccaagaacacgctgtatctgctaatgaacagcctgagagccgaggacacggctgtgtattactgtgcgaggtcagtggctggttaccactactactacggtatggacgtctggggccaagggaccacggtcaccgtctcctca

SEQ ID NO: 431 - protein, 122 aa, Homo sapiens
QVQLVESGGGVVQSGRSLRLSCAASGFTFRNYGMHWVRQAPGKGLEWVAVIWFDGSNKYYADSVKGRSTISRDNSKNTLYLLMNSLRAEDTAVYYCARSVAGYHYYYGMDVWGQGTTVTVSS

SEQ ID NO: 432 - DNA, 324 bp, Homo sapiens
tcttctgagctgactcaggaccctgctgtgtctgtggccttgggacagacagtcaggatcacatgccagggagacagcctcagaagctattatgcaagctggtaccagcagaagccaagacaggcccctgtacttgtcatctatggtaaaaacaaccggccctcagggatcccagaccgaatctctggctccacctcaggaaacacagcttccttgaccatcactggggctcaggcggaagatgaggctgactattactgtaaatcccgggacatcattggtgaccatctggtgttcggcggagggaccaaactgaccgtccta

SEQ ID NO: 433 - protein, 108 aa, Homo sapiens
SSELTQDPAVSVALGQTVRITCQGDSLRSYYASWYQQKPRQAPVLVIYGKNNRPSGIPDRISGSTSGNTASLTITGAQAEDEADYYCKSRDIIGDHLVFGGGTKLTVL

SEQ ID NO: 434 - DNA, 342 bp, Homo sapiens
caggtgcagctggtggagtctgggggaggcgtggtccagcctgggaggtccctgagactctcctgtgcagcgtctggattcaccttcagtagctatggcatgcactgggtccgccaggctccaggcaaggggctggagtgggtggcagttatatggtatgatggaagtaataaatactatgcagactccgtgaagggccgattcaccatctccagagacaattccaagaacacgctgtatctgcaaatgaacagcctgagagccgaggacacggctgtgtattactgtgtgagagatcggggactggactggggccagggaaccctggtcaccgtctcctca

SEQ ID NO: 435 - protein, 114 aa, Homo sapiens
QVQLVESGGGVVQPGRSLRLSCAASGFTFSSYGMHWVRQAPGKGLEWVAVIWYDGSNKYYADSVKGRFTISRDNSKNTLYLQMNSLRAEDTAVYYCVRDRGLDWGQGTLVTVSS

SEQ ID NO: 436 - DNA, 324 bp, Homo sapiens
tcttctgagctgactcaggaccctgctgtgtctgtggccttgggacagacagtcaggatcacatgccaaggagacagcctcagaggctattatgcaagctggtaccagcagaagccaagacaggcccctgtacttgtcatctatggtaaaaacaaccggccctcagggatcccagaccgattctctggctccacctcaggaaacacagcttccttgaccatcactggggctcaggcggaagatgaggctgactattactgtaagtcccgggacagcagtggtgaccatctggtgttcggcggagggaccaagctgaccgtccta

SEQ ID NO: 437 - protein, 108 aa, Homo sapiens
SSELTQDPAVSVALGQTVRITCQGDSLRGYYASWYQQKPRQAPVLVIYGKNNRPSGIPDRFSGSTSGNTASLTITGAQAEDEADYYCKSRDSSGDHLVFGGGTKLTVL

SEQ ID NO: 438 - DNA, 366 bp, Homo sapiens
caggtgcaggtggtggagtctgggggaggcgtggtccagcctggggggtccctgagactctcctgtgcagcgtctggattcaccttcagtaactatggcatgcactgggtccgccaggctccaggcaaggggctggagtgggtggcagttatttggtatgatggaagtagtaaatactatgcagactccgtgaagggccgatccaccatctccagagacaattccaagaacacggtgtatctgcaaatgaacagcctgagagccgaggacacggctgtgtattactgtgcgaggtcagtggctggttaccactactactacggtatggacgtctggggccaagggaccacggtcaccgtctcctca

SEQ ID NO: 439 - protein, 122 aa, Homo sapiens
QVQVVESGGGVVQPGGSLRLSCAASGFTFSNYGMHWVRQAPGKGLEWVAVIWYDGSSKYYADSVKGRSTISRDNSKNTVYLQMNSLRAEDTAVYYCARSVAGYHYYYGMDVWGQGTTVTVSS

SEQ ID NO: 440 - DNA, 324 bp, Homo sapiens; identical to SEQ ID NO: 436

SEQ ID NO: 441 - protein, 108 aa, Homo sapiens; identical to SEQ ID NO: 437

SEQ ID NO: 442 - DNA, 366 bp, Homo sapiens
caggtgcagctggtggagtctgggggaggcgtggtccagcctgggaggtccctgagtctctcctgtgcagcgtctggattcaccttcagtagctatggcatgcactgggtccgccaggctccaggcaaggggctggagtgggtggcagttatatggtatgatggaagttataaagactatgcagactccgtgaagggccgatccaccatctccagagacaactccaagaacacgctgtatctgcaaatgaacagcctgagagccgaggacacggctgtgtattattgtgcgaggtcagtggctggttaccactactactacggtatggacgtctggggccaagggaccacggtcaccgtctcctca

SEQ ID NO: 443 - protein, 122 aa, Homo sapiens
QVQLVESGGGVVQPGRSLSLSCAASGFTFSSYGMHWVRQAPGKGLEWVAVIWYDGSYKDYADSVKGRSTISRDNSKNTLYLQMNSLRAEDTAVYYCARSVAGYHYYYGMDVWGQGTTVTVSS

SEQ ID NO: 444 - DNA, 324 bp, Homo sapiens
tcttctgagctgactcaggaccctgctgtgtctgtggccttgggacagacagtcaggatcacatgccaaggagacagcctcagaacctattatgcaagctggtaccagcagaagccaagacaggcccctattcttgtcatctatggtaaaaacaaccggccctcagggatcccagaccgattctctggctccacctcaggaatcacagcttccttgaccatcactggggctcaggcggaagatgaggctgactattactgtaaatcccgggacatcattggtaaccatctgctgttcggcggagggactaagctgaccgtccta

SEQ ID NO: 445 - protein, 108 aa, Homo sapiens
SSELTQDPAVSVALGQTVRITCQGDSLRTYYASWYQQKPRQAPILVIYGKNNRPSGIPDRFSGSTSGITASLTITGAQAEDEADYYCKSRDIIGNHLLFGGGTKLTVL

SEQ ID NO: 446 - DNA, 375 bp, Homo sapiens
caggtgcagctggtggcgtctgggggaggcgtggtccagcctgggaggtccctgagactctcctgtgcagcgtctggattcaccctcagtagctatggcatgcactgggtccgccaggctccaggccaggggctggagtgggtggcagtcatatggtatgatggaagtaacaaatactatgcagcctccgtgaagggccgattcaccatctccagagacaattccaagaacacgctgtatctgcaaatgaacagtctgagagccgaggacacggctgtgtattactgtgcgagagggggtggttcggggagtcatcgctactactactacggtatggacgtctggggccaagggaccacggtcaccgtctcctca

SEQ ID NO: 447 - protein, 125 aa, Homo sapiens
QVQLVASGGGVVQPGRSLRLSCAASGFTLSSYGMHWVRQAPGQGLEWVAVIWYDGSNKYYAASVKGRFTISRDNSKNTLYLQMNSLRAEDTAVYYCARGGGSGSHRYYYYGMDVWGQGTTVTVSS

SEQ ID NO: 448 - DNA, 324 bp, Homo sapiens; identical to SEQ ID NO: 444

SEQ ID NO: 449 - protein, 108 aa, Homo sapiens; identical to SEQ ID NO: 445

SEQ ID NO: 450 - DNA, 366 bp, Homo sapiens
caggtgcaagtggtggagtctgggggaggcgtggtccagcctgggaggtccctgagactctcctgtgcagcgtctggattcaccttcagtaactatggcatgcactgggtccgccaggctccaggcaaggggctggagtgggtggcagttatatggtatgatggaggtaataaatactatgcagactccgtgaagggccgatccatcatctccagagacaattccaagagcacgctgtatctgcaaatgaacagcctgagagccgaggacacggctgtttattattgtgcgaggtcagtggctggttaccattattactacggtatggacgtctggggccaagggaccacggtcaccgtcgcctca

SEQ ID NO: 451 - protein, 122 aa, Homo sapiens
QVQVVESGGGVVQPGRSLRLSCAASGFTFSNYGMHWVRQAPGKGLEWVAVIWYDGGNKYYADSVKGRSIISRDNSKSTLYLQMNSLRAEDTAVYYCARSVAGYHYYYGMDVWGQGTTVTVAS

SEQ ID NO: 452 - DNA, 327 bp, Homo sapiens
cagtctgccctgactcagcctgcctccgtgtctgggtctcctggacagtcgatcaccatctcctgcactggaaccagcagtgacgttggtggttataactctgtctcctggtaccaacagcacccaggcaaaccccccaaactcatgatttatgaggtcagtaatcggccctcagggatttctaatcgcttctctggctccaagtctggcaacacggcctccctgaccatctctgggctccaggctgaggacgaggctgattatttctgcagctcatatacaagcaccagcatggtcttcggcggagggaccaagctggccgtccta

SEQ ID NO: 453 - protein, 109 aa, Homo sapiens
QSALTQPASVSGSPGQSITISCTGTSSDVGGYNSVSWYQQHPGKPPKLMIYEVSNRPSGISNRFSGSKSGNTASLTISGLQAEDEADYFCSSYTSTSMVFGGGTKLAVL

SEQ ID NO: 454 - DNA, 366 bp, Homo sapiens; identical to SEQ ID NO: 450

SEQ ID NO: 455 - protein, 122 aa, Homo sapiens; identical to SEQ ID NO: 451

SEQ ID NO: 456 - DNA, 324 bp, Homo sapiens
tcttctgagctgactcaggaccctgctgtgtctgtggccttgggacagacagtcaggatcacatgccaaggagacagcctcagaggctattatgcaagctggtaccagcagaagccaagacaggcccctgtacttgtcatctatggtaaaaacaaccggccctcagggatcccagaccgattctctggctccacgtcaggaaacacagcttccttgaccatcactggggctcaggcggaagatgaggctgactattactgtaactcccgggacaacattggtgaccatctggtgttcggcggagggaccaagctgaccgtccta

SEQ ID NO: 457 - protein, 108 aa, Homo sapiens
SSELTQDPAVSVALGQTVRITCQGDSLRGYYASWYQQKPRQAPVLVIYGKNNRPSGIPDRFSGSTSGNTASLTITGAQAEDEADYYCNSRDNIGDHLVFGGGTKLTVL

SEQ ID NO: 458 - DNA, 381 bp, Homo sapiens
gaggtgcagctggtggagtctgggggaggcttggtccagcctggggggtccctgagactctcctgtgcagcctccggattcacctttagtagctattggatgagctgggtccgccaggctccagggaaggggctggagtgggtggccagcataaaacaagatggaagtgagaaatactatgtggactctgtgaagggccgattcaccatctccagagacaacgccaggaactcactgtatctgcaaatgaacagcctgagagccgaggacacggctgtgtattactgtgcgagagatcttgtattaatggtgtatgatatagactactactactacggtatggacgtctggggccaagggaccacggtcaccgtctcctca

SEQ ID NO: 459 - protein, 127 aa, Homo sapiens
EVQLVESGGGLVQPGGSLRLSCAASGFTFSSYWMSWVRQAPGKGLEWVASIKQDGSEKYYVDSVKGRFTISRDNARNSLYLQMNSLRAEDTAVYYCARDLVLMVYDIDYYYYGMDVWGQGTTVTVSS

SEQ ID NO: 460 - DNA, 336 bp, Homo sapiens
gatattgtgatgactcagtctccactctccctgcccgtcacccctggagagccggcctccatctcctgcaggtctagtcagagcctcctgcatagtaatggatacaactatttggattggtacctgcagaagccagggcagtctccacagctcctgatctatttgggttctaatcgggcctccggggtccctgacaggttcagtggcagtggatcaggcacagattttacactgaaaatcagcagagtggaggctgaggatgttggggtttattactgcatgcaagctctacaaactccgctcactttcggcggagggaccaaggtagagatcaaa

SEQ ID NO: 461 - protein, 112 aa, Homo sapiens
DIVMTQSPLSLPVTPGEPASISCRSSQSLLHSNGYNYLDWYLQKPGQSPQLLIYLGSNRASGVPDRFSGSGSGTDFTLKISRVEAEDVGVYYCMQALQTPLTFGGGTKVEIK

SEQ ID NO: 462 - DNA, 381 bp, Homo sapiens
gaggtgcagctggtggagtctgggggaggcttggtccagcctggggggtccctgagactctcctgtgcagcctccggattcacctttagtaactattggatgagctgggtccgccaggctccagggaaggggctggagtgggtggccagcataaaacaagatggaagtgagaaatactatgtggactctgtgaagggccgattcgccatctccagagacaacgccaagaactcactgtttctgcaaatgaacagcctgagagccgaggacacggctgtgtattactgtgcgagagatcttgtactaatggtgtatgatatagactactactactacggtatggacgtctggggccaagggaccacggtcaccgtctcctca

SEQ ID NO: 463 - protein, 127 aa, Homo sapiens
EVQLVESGGGLVQPGGSLRLSCAASGFTFSNYWMSWVRQAPGKGLEWVASIKQDGSEKYYVDSVKGRFAISRDNAKNSLFLQMNSLRAEDTAVYYCARDLVLMVYDIDYYYYGMDVWGQGTTVTVSS

SEQ ID NO: 464 - DNA, 336 bp, Homo sapiens
gatattgtgatgactcagtctccactctccctgcctgtcacccctggagagccggcctccatctcttgcaggtctagtcagagcctcctgcatagtaatgggtacaactatttggattggtacctgcagaagccagggcagtctccacagctcctgatctatttgggttctaatcgggcctccggggtccctgacaggttcagtggcagtggatcaggcacacatcttacactgaaaatcagcagagtggaggctgaggatgttggagtttattactgcatgcaaactctacaaactccgctcactttcggcggagggaccaaggtggagatcaaa

SEQ ID NO: 465 - protein, 112 aa, Homo sapiens
DIVMTQSPLSLPVTPGEPASISCRSSQSLLHSNGYNYLDWYLQKPGQSPQLLIYLGSNRASGVPDRFSGSGSGTHLTLKISRVEAEDVGVYYCMQTLQTPLTFGGGTKVEIK

SEQ ID NO: 466 - DNA, 342 bp, Homo sapiens
caggtgcagctggtggagtctgggggaggcgtggcccagcctgggaggtccctgagactctcctgtgcagcgtctggattcaccttcagtagctatggcatgcactgggtccgccaggctccaggcaaggggctggagtgggtggcagttatatactatgatggaattaataaacactatgcagactccgtgaagggccgattcaccatctccagagacaattccaagaacacgctgtatctgcaaatgaacagcctgagagccgaggacacggctgtgtattactgtgcgagagatcggggactggactggggccagggaaccctggtcaccgtctcctca

SEQ ID NO: 467 - protein, 114 aa, Homo sapiens
QVQLVESGGGVAQPGRSLRLSCAASGFTFSSYGMHWVRQAPGKGLEWVAVIYYDGINKHYADSVKGRFTISRDNSKNTLYLQMNSLRAEDTAVYYCARDRGLDWGQGTLVTVSS

SEQ ID NO: 468 - DNA, 339 bp, Homo sapiens
gacatcgtgatgacccagtctccagactccctggctgtgtctctgggcgagagggccaccatcaactgcaagtccagccagagtgttttatacagctccaacagtaagaactacttagtttggtaccagcagaaaccaggacagcctcctaagctgctcatttactgggcctctacccgggaatccggggtccctgaccgattcagtggcagcgggtctgggacagatttcactctcaccatcagcagcctgcaggctgaagatgtggcagtttattactgtcaacaatattatagtactccgtggacgttcggccaagggaccaaggtggaaatcaaa

SEQ ID NO: 469 - protein, 113 aa, Homo sapiens
DIVMTQSPDSLAVSLGERATINCKSSQSVLYSSNSKNYLVWYQQKPGQPPKLLIYWASTRESGVPDRFSGSGSGTDFTLTISSLQAEDVAVYYCQQYYSTPWTFGQGTKVEIK

SEQ ID NO: 470 - DNA, 357 bp, Homo sapiens
gaggtgcagctggtggagtctgggggaggcttggtccagcctggggggtccctgagactctcctgtgcagcctctggactcacctttagtaacttttggatgagctgggtccgccaggctccagggaaggggctggagtgggtggccaacataaagcaagatggaaatgataaatactatgtggactctgtgaagggccgattcaccatctccagagacaacgccaagaattcactgtatctgcaaatgaacagcctgagagccgaggacacggctgtgtattactgtgcgagagagtcaaactggggatttgcttttgatatctggggccaagggacaatggtcaccgtctcttca

SEQ ID NO: 471 - protein, 119 aa, Homo sapiens
EVQLVESGGGLVQPGGSLRLSCAASGLTFSNFWMSWVRQAPGKGLEWVANIKQDGNDKYYVDSVKGRFTISRDNAKNSLYLQMNSLRAEDTAVYYCARESNWGFAFDIWGQGTMVTVSS

SEQ ID NO: 472 - DNA, 327 bp, Homo sapiens; identical to SEQ ID NO: 145

SEQ ID NO: 473 - protein, 109 aa, Homo sapiens; identical to SEQ ID NO: 33

SEQ ID NO: 474 - DNA, 357 bp, Homo sapiens
gaggtgcagctggtggagtctgggggaggtttggtccagcctggggggtccctgagactctcctgtgcagcctctggactcacctttagtaacttttggatgagctgggtccgccaggctccagggaaggggctggagtgggtggccaacataaagcaagatggaagtgagaaatactatgtggactctgtgaagggccgattcaccatctccagagacaacgccaagaattcactgtatctgcaaatgaacagcctgagagccgaggacacggctgtgtattactgtgcgagagagtcaaactggggatttgcttttgatatctggggccaagggacaatggtcaccgtctcttca

SEQ ID NO: 475 - protein, 119 aa, Homo sapiens
EVQLVESGGGLVQPGGSLRLSCAASGLTFSNFWMSWVRQAPGKGLEWVANIKQDGSEKYYVDSVKGRFTISRDNAKNSLYLQMNSLRAEDTAVYYCARESNWGFAFDIWGQGTMVTVSS

SEQ ID NO: 476 - DNA, 327 bp, Homo sapiens
cagtctgtgctgactcagccaccctcagcgtctgggacccccgggcagagggtcaccatctcttgttctggaagcagctccaacatcggaagtaaaactgtaaactggtaccagcagttcccaggaacggcccccaaactcctcatctatagtaataatcggcggccctcaggggtccctgaccgattctctggctccaagtctggcacctcagcctccctggccatcagtgggctccagtctgaggatgaggctgattattactgtgcaacatgggatgacagactgaattgggtgttcggcgcagggaccaagctgaccgtccta

SEQ ID NO: 477 - protein, 109 aa, Homo sapiens
QSVLTQPPSASGTPGQRVTISCSGSSSNIGSKTVNWYQQFPGTAPKLLIYSNNRRPSGVPDRFSGSKSGTSASLAISGLQSEDEADYYCATWDDRLNWVFGAGTKLTVL

SEQ ID NO: 478 - DNA, 366 bp, Homo sapiens
caggtcaccttgaaggagtctggtcctgtgctggtgaaacccacagagaccctcacgctgacctgcaccgtctctgggttctcactcagcaatgttagaatgggtgtgagctggatccgtcagcccccagggaaggccctggagtggcttgcacacattttttcgaatgacgaaaattcctacagaacatctctgaagagcaggctcaccatctccaaggacacctccaaaagccaggtggtccttaccatgaccaacatggaccctgtggacacagccacatattactgtgcacggatagtgggagctacaacggatgatgcttttgatatctggggccaagggacaatggtcaccgtctcttca

SEQ ID NO: 479 - protein, 122 aa, Homo sapiens
QVTLKESGPVLVKPTETLTLTCTVSGFSLSNVRMGVSWIRQPPGKALEWLAHIFSNDENSYRTSLKSRLTISKDTSKSQVVLTMTNMDPVDTATYYCARIVGATTDDAFDIWGQGTMVTVSS

SEQ ID NO: 480 - DNA, 324 bp, Homo sapiens
tcctatgtgctgactcagccaccctcggtgtcagtggccccaggacagacggccaggattacctgtgggggaaacaacattggaagtaaaagtgtgcactggtaccagcagaagccaggccaggcccctgtgctggtcgtctatgatgatagcgaccggccctcagggatccctgagcgattctctggctccaactctgggaacacggccaccctgaccatcagcagggtcgaagccggggatgaggccgacttttactgtcaggtgtgggatagtagtagtgatcctgtggtattcggcggagggaccaagctgaccgtccta

SEQ ID NO: 481 - protein, 108 aa, Homo sapiens
SYVLTQPPSVSVAPGQTARITCGGNNIGSKSVHWYQQKPGQAPVLVVYDDSDRPSGIPERFSGSNSGNTATLTISRVEAGDEADFYCQVWDSSSDPVVFGGGTKLTVL

SEQ ID NO: 482 - DNA, 381 bp, Homo sapiens
gaggtgcagctggtggagtctgggggaggcttggtccagcctggggggtccctgagactctcctgtgcagcctctggattcacctttagtaactattggatgacctgggtccgccaggctccagggaaggggctggagtgggtggccagcataaagcaagatggaagtgagagatactatgtggactctgtgaagggccgattcaccatctcccgagacaccgccaagaactctctgtatctccaaatgaacagcctgcgagccgaggacacggctgtgtattactgtgcgagacctcttgtactaatggtgtatgctctacactactactactacggtatggacgtctggggccacgggaccacggtcaccgtctcctca

SEQ ID NO: 483 - protein, 127 aa, Homo sapiens
EVQLVESGGGLVQPGGSLRLSCAASGFTFSNYWMTWVRQAPGKGLEWVASIKQDGSERYYVDSVKGRFTISRDTAKNSLYLQMNSLRAEDTAVYYCARPLVLMVYALHYYYYGMDVWGHGTTVTVSS

SEQ ID NO: 484 - DNA, 336 bp, Homo sapiens
gatattgtgatgactcagtctccactctccctgcccgtcacccctggagagccggcctccatctcctgcaggtctagtcagagcctcctgcatagtaatggatacaactatttggattggtacctgcagaagccagggcagtctccacagctcctgatctatttgggttctaatcgggcctccggggtccctgacaggttcagtggcagtggatcaggcacagattttacactgaaaatcagcagagtggaggctgaggatgttggggtttattactgcatgcaagctctacaaactccgctcactttcggcggagggaccaaggtggagatcaaa

SEQ ID NO: 485 - protein, 112 aa, Homo sapiens; identical to SEQ ID NO: 461

SEQ ID NO: 486 - protein, 100 aa, Homo sapiens
QVTLKESGPVLVKPTETLTLTCTVSGFSLSNARMGVSWIRQPPGKALEWLAHIFSNDEKSYSTSLKSRLTISKDTSKSQVVLTMTNMDPVDTATYYCARI

SEQ ID NO: 487 - protein, 98 aa, Homo sapiens
EVQLVESGGGLVQPGGSLRLSCAASGFTFSSYWMSWVRQAPGKGLEWVANIKQDGSEKYYVDSVKGRFTISRDNAKNSLYLQMNSLRAEDTAVYYCAR

SEQ ID NO: 488 - protein, 98 aa, Homo sapiens
QVQLVESGGGVVQPGRSLRLSCAASGFTFSSYGMHWVRQAPGKGLEWVAVIWYDGSNKYYADSVKGRFTISRDNSKNTLYLQMNSLRAEDTAVYYCAR

SEQ ID NO: 489 - protein, 93 aa, Homo sapiens
DIVMTQSPLSLPVTPGEPASISCRSSQSLLHSNGYNYLDWYLQKPGQSPQLLIYLGSNRASGVPDRFSGSGSGTDFTLKISRVEAEDVGVYYC

SEQ ID NO: 490 - protein, 94 aa, Homo sapiens
DIVMTQSPDSLAVSLGERATINCKSSQSVLYSSNNKNYLAWYQQKPGQPPKLLIYWASTRESGVPDRFSGSGSGTDFTLTISSLQAEDVAVYYC

SEQ ID NO: 491 - protein, 89 aa, Homo sapiens
QSVLTQPPSASGTPGQRVTISCSGSSSNIGSNTVNWYQQLPGTAPKLLIYSNNQRPSGVPDRFSGSKSGTSASLAISGLQSEDEADYYC

SEQ ID NO: 492 - protein, 87 aa, Homo sapiens
SYVLTQPPSVSVAPGKTARITCGGNNIGSKSVHWYQQKPGQAPVLVIYYDSDRPSGIPERFSGSNSGNTATLTISRVEAGDEADYYC

SEQ ID NO: 493 - protein, 49 aa, Homo sapiens
QVQLVQSGAEVKKPGASVKVSCKASGYTFTGYYMHWVRQAPGQGLEWMG

SEQ ID NO: 494 - protein, 98 aa, Homo sapiens; identical to SEQ ID NO: 488

SEQ ID NO: 495 - protein, 98 aa, Homo sapiens; identical to SEQ ID NO: 488

SEQ ID NO: 496 - protein, 88 aa, Homo sapiens
DIQMTQSPSSLSASVGDRVTITCRASQGISNYLAWYQQKPGKVPKLLIYAASTLQSGVPSRFSGSGSGTDFTLTISSLQPEDVATYYC

SEQ ID NO: 497 - protein, 90 aa, Homo sapiens
QSALTQPASVSGSPGQSITISCTGTSSDVGGYNYVSWYQQHPGKAPKLMIYEVSNRPSGVSNRFSGSKSGNTASLTISGLQAEDEADYYC

SEQ ID NO: 498 - protein, 87 aa, Homo sapiens
SSELTQDPAVSVALGQTVRITCQGDSLRSYYASWYQQKPGQAPVLVIYGKNNRPSGIPDRFSGSSSGNTASLTITGAQAEDEADYYC

SEQ ID NO: 499 - protein, 13 aa, Homo sapiens
SGSSSNIGSKTVN